European Patent Specification EP 3 699 930 B1, published February 7, 2024. Title: COMPUTATIONAL ANALYSIS OF BIOLOGICAL DATA USING MANIFOLD AND A HYPERPLANE. Applicant: MEMED DIAGNOSTICS LTD. EDEN, Eran OVED, Kfir NAVON, Roy COHEN-DOTAN, Assaf BOICO, Olga. The sequence listing filed with the application follows.

SEQUENCE LISTING (38 sequences)

SEQ ID NO: 1 - DNA, 1953 bp, Homo sapiens
acagaacccagaaaaacaactcattcgctttcatttcctcactgactataaaagaatagagaaggaagggcttcagtgaccggctgcctggctgacttacagcagtcagactctgacaggatcatggctatgatggaggtccaggggggacccagcctgggacagacctgcgtgctgatcgtgatcttcacagtgctcctgcagtctctctgtgtggctgtaacttacgtgtactttaccaacgagctgaagcagatgcaggacaagtactccaaaagtggcattgcttgtttcttaaaagaagatgacagttattgggaccccaatgacgaagagagtatgaacagcccctgctggcaagtcaagtggcaactccgtcagctcgttagaaagatgattttgagaacctctgaggaaaccatttctacagttcaagaaaagcaacaaaatatttctcccctagtgagagaaagaggtcctcagagagtagcagctcacataactgggaccagaggaagaagcaacacattgtcttctccaaactccaagaatgaaaaggctctgggccgcaaaataaactcctgggaatcatcaaggagtgggcattcattcctgagcaacttgcacttgaggaatggtgaactggtcatccatgaaaaagggttttactacatctattcccaaacatactttcgatttcaggaggaaataaaagaaaacacaaagaacgacaaacaaatggtccaatatatttacaaatacacaagttatcctgaccctatattgttgatgaaaagtgctagaaatagttgttggtctaaagatgcagaatatggactctattccatctatcaagggggaatatttgagcttaaggaaaatgacagaatttttgtttctgtaacaaatgagcacttgatagacatggaccatgaagccagtttttttggggcctttttagttggctaactgacctggaaagaaaaagcaataacctcaaagtgactattcagttttcaggatgatacactatgaagatgtttcaaaaaatctgaccaaaacaaacaaacagaaaacagaaaacaaaaaaacctctatgcaatctgagtagagcagccacaaccaaaaaattctacaacacacactgttctgaaagtgactcacttatcccaagagaatgaaattgctgaaagatctttcaggactctacctcatatcagtttgctagcagaaatctagaagactgtcagcttccaaacattaatgcaatggttaacatcttctgtctttataatctactccttgtaaagactgtagaagaaagagcaacaatccatctctcaagtagtgtatcacagtagtagcctccaggtttccttaagggacaacatccttaagtcaaaagagagaagaggcaccactaaaagatcgcagtttgcctggtgcagtggctcacacctgtaatcccaacattttgggaacccaaggtgggtagatcacgagatcaagagatcaagaccatagtgaccaacatagtgaaaccccatctctactgaaagtacaaaaattagctgggtgtgttggcacatgcctgtagtcccagctacttgagaggctgaggcaagagaattgtttgaacccgggaggcagaggttgcagtgtggtgagatcatgccactacactccagcctggcgacagagcgagacttggtttcaaaaaaaaaaaaaaaaaaaacttcagtaagtacgtgttatttttttcaataaaattctattacagtatgtcatgtttgctgtagtgctcatatttattgttgtttttgttttagtactcacttgtttcataatatcaagattactaaaaatgggggaaaagacttctaatctttttttcataatatctttgacacatattacagaagaaataaatttcttacttttaatttaatatga

SEQ ID NO: 2 - DNA, 1805 bp, Homo sapiens
acagaacccagaaaaacaactcattcgctttcatttcctcactgactataaaagaatagagaaggaagggcttcagtgaccggctgcctggctgacttacagcagtcagactctgacaggatcatggctatgatggaggtccaggggggacccagcctgggacagacctgcgtgctgatcgtgatcttcacagtgctcctgcagtctctctgtgtggctgtaacttacgtgtactttaccaacgagctgaagcagatgcaggacaagtactccaaaagtggcattgcttgtttcttaaaagaagatgacagttattgggaccccaatgacgaagagagtatgaacagcccctgctggcaagtcaagtggcaactccgtcagctcgttagaaagactccaagaatgaaaaggctctgggccgcaaaataaactcctgggaatcatcaaggagtgggcattcattcctgagcaacttgcacttgaggaatggtgaactggtcatccatgaaaaagggttttactacatctattcccaaacatactttcgatttcaggaggaaataaaagaaaacacaaagaacgacaaacaaatggtccaatatatttacaaatacacaagttatcctgaccctatattgttgatgaaaagtgctagaaatagttgttggtctaaagatgcagaatatggactctattccatctatcaagggggaatatttgagcttaaggaaaatgacagaatttttgtttctgtaacaaatgagcacttgatagacatggaccatgaagccagtttttttggggcctttttagttggctaactgacctggaaagaaaaagcaataacctcaaagtgactattcagttttcaggatgatacactatgaagatgtttcaaaaaatctgaccaaaacaaacaaacagaaaacagaaaacaaaaaaacctctatgcaatctgagtagagcagccacaaccaaaaaattctacaacacacactgttctgaaagtgactcacttatcccaagagaatgaaattgctgaaagatctttcaggactctacctcatatcagtttgctagcagaaatctagaagactgtcagcttccaaacattaatgcaatggttaacatcttctgtctttataatctactccttgtaaagactgtagaagaaagagcaacaatccatctctcaagtagtgtatcacagtagtagcctccaggtttccttaagggacaacatccttaagtcaaaagagagaagaggcaccactaaaagatcgcagtttgcctggtgcagtggctcacacctgtaatcccaacattttgggaacccaaggtgggtagatcacgagatcaagagatcaagaccatagtgaccaacatagtgaaaccccatctctactgaaagtacaaaaattagctgggtgtgttggcacatgcctgtagtcccagctacttgagaggctgaggcaagagaattgtttgaacccgggaggcagaggttgcagtgtggtgagatcatgccactacactccagcctggcgacagagcgagacttggtttcaaaaaaaaaaaaaaaaaaaacttcagtaagtacgtgttatttttttcaataaaattctattacagtatgtcatgtttgctgtagtgctcatatttattgttgtttttgttttagtactcacttgtttcataatatcaagattactaaaaatgggggaaaagacttctaatctttttttcataatatctttgacacatattacagaagaaataaatttcttacttttaatttaatatga

SEQ ID NO: 3 - DNA, 1334 bp, Homo sapiens
atttcctcactgactataaaagaatagagaaggaagggcttcagtgaccggctgcctggctgacttacagcagtcagactctgacaggatcatggctatgatggaggtccaggggggacccagcctgggacagacctgcgtgctgatcgtgatcttcacagtgctcctgcagtctctctgtgtggctgtaacttacgtgtactttaccaacgagctgaagcagtttgcagaaaatgattgccagagactaatgtctgggcagcagacagggtcattgctgccatcttgaagtctaccttgctgagtctaccctgctgacctcaagccccatcaaggactggttgaccctggcctagacaaccaccgtgtttgtaacagcaccaagagcagtcaccatggaaatccacttttcagaaccaagggcttctggagctgaagaacaggcacccagtgcaagagctttcttttcagaggcacgcaaatgaaaataatccccacacgctaccttctgcccccaatgcccaagtgtggttagttagagaatatagcctcagcctatgatatgctgcaggaaactcatattttgaagtggaaaggatgggaggaggcgggggagacgtatcgtattaattatcattcttggaataaccacagcacctcacgtcaacccgccatgtgtctagtcaccagcattggccaagttctataggagaaactaccaaaattcatgatgcaagaaacatgtgagggtggagagagtgactggggcttcctctctggatttctattgttcagaaatcaatatttatgcataaaaaggtctagaaagagaaacaccaaaatgacaatgtgatctctagatggtatgattatgggtactttttttcctttttatttttctatattttacaaattttctacagggaatgttataaaaatatccatgctatccatgtataattttcatacagatttaaagaacacagcatttttatatagtcttatgagaaaacaaccatactcaaaattatgcacacacacagtctgatctcacccctgtaaacaagagatatcatccaaaggttaagtaggaggtgagaatatagctgctattagtggttgttttgttttgtttttgtgatttacttatttagtttttggagggttttttttttcttttagaaaagtgttctttacttttccatgcttccctgcttgcctgtgtatcctgaatgtatccaggctttataaactcctgggtaataatgtagctacattaacttgttaacctcccatccacttatacccaggaccttactcaattttccaggttc

SEQ ID NO: 4 - protein, 281 aa, Homo sapiens [sequence omitted]

SEQ ID NO: 5 - protein, 101 aa, Homo sapiens
MAMMEVQGGPSLGQTCVLIVIFTVLLQSLCVAVTYVYFTNELKQMQDKYSKSGIACFLKEDDSYWDPNDEESMNSPCWQVKWQLRQLVRKTPRMKRLWAAK

SEQ ID NO: 6 - protein, 65 aa, Homo sapiens
MAMMEVQGGPSLGQTCVLIVIFTVLLQSLCVAVTYVYFTNELKQFAENDCQRLMSGQQTGSLLPS

SEQ ID NO: 7 - protein, 223 aa, Homo sapiens
QDHGYDGGPGGTQPGTDLRADRDLHSAPAVSLCGCNLRVLYQRAEAEKQQNISPLVRERGPQRVAAHITGTRGRSNTLSSPNSKNEKALGRKINSWESSRSGHSFLSNLHLRNGELVIHEKGFYYIYSQTYFRFQEEIKENTKNDKQMVQYIYKYTSYPDPILLMKSARNSCWSKDAEYGLYSIYQGGIFELKENDRIFVSVTNEHLIDMDHEASFFGAFLVG

SEQ ID NO: 8 - protein, 178 aa, Homo sapiens
KEKQQNISPLVRERGPQRVAAHITGTRGRSNTLSSPNSKNEKALGRKINSWESSRSGHSFLSNLHLRNGELVIHEKGFYYIYSQTYFRFQEEIKENTKNDKQMVQYIYKYTSYPDPILLMKSARNSCWSKDAEYGLYSIYQGGIFELKENDRIFVSVTNEHLIDMDHEASFFGAFLVG

SEQ ID NO: 9 - DNA, 2421 bp, Homo sapiens
caccctcatgagccccgggtacgtttaactattgagggccaggaaattgccttcctcctggacactggcgcagccttctcagggttaatctcctgtcctggatgactgtcttcaaggtccgttaccacccgaggaatcctgggacagcctataaccaggtatttctcccacatcctcagttgtaattgagagactttaatcttttcacatgccttttttgttattcctgaaagtcccacacccttattaaggagggatatattagccaaggctggagctattatctacatgaatatggggaaaaagttacccatttgctgtcccctacttgaggagggaatcaaccctgaagtctgggcattggaaggacaatttggaagggcaaaaaatgcctgcccagtccaaatcaggttaaaagatcccaccacttttccgtatcaaaggcaatatcccttaaggcctgaagctcataaaggattatagaatattgttaaacatttaaaagctcaaggcttagtgaggaaatgcagcagtccctgcaacaccccagttctaggagtacaaaaaccaaacagtcagtggagactagtgcaagatcttagactcattaatgaggcagtaattcctctatatccagttgtacccaacccctataccctgctctctcaaataccaggggaagcagaatggttcacggttctggacctcaaggatgccttcttctttattcccctgcactctgactcccagtttctctttgcttttgaggatcccacagaccacacgtcccaacttacacagatggtcttgccccaagggtttagggatagccctcatctgtttggtcaggcactggcccaagatctataggccacttctcaagtccaggcactctggtccttcaatatgtggatgatttacttttggctaccagtttggaagcctcgtgccagcaggctactctggatctcttgaactttctggctaatcaagggtacaaggtgtctaggtcgaaggcccagctttgcctacagcaggttaaatatctaagcctaatcttagccaaagggaccagggccctcagcaaggaatgaatacagcctatactggcttatcctcaccctaagacattaaaacagttgcggggattccttggaattactggcttttgctgactatggatctccagatacagcgagacagccaggcccctctatactctaatcaaggaaacccagagggcaaatactcatctagtcgaaagggaaccagaggcagaaacagccttcaaaagcttaaagcaggctctagtacaagctccagctttaagccttcccacaggacagaacttctctttatacatcacagagagagccaagatagctcttggagtccttagactcgtgggacaaccccacaaccagtggcatacctaagtaaggaaattgatgtagtagcaaaaggctggcctcactgtttaagggtagttgcagcagcggccgtcttagcgtcagaggctatcagaataatacaaggaaaggatctcactgtctggactactcatgatgtaaatggcatactaggtgccaaaggaagtttatggctatcagacaaccgcctcttagatgccaggcactactccttgagggactggtgcttaaaatatgcacgtgcgtggccctcaaccctgccacttttctcccagaggatggggaaccaattgagcatgactgccaacaaattatagtccagacttatgccgcccgagatgatctcttagaagtccccttaactaatcctgaccttaacctatataccgacggaagttcatttgtggagaatgggatacgaagggcaggttacgccatagtgatgtaaccacacttgaaagcaagcctcttcccccagggaccagtgcccagttagcagaactagtggcacttacccgagccttagaactgggaaagggaaaaagaataaatgtgtatacagataacaagtatgcttatctaatcctacatgcccatgctgcaatatggaaagaatgggagttcctaacctctgggaacccccgctggatgccacagggaagttatggagttattgcacatggtgcaggaacccaaagaggtgggagtcttacactaccaaggccatcaaaatgggaaggagaggggagaacagcagcataagcggctggcagaggtagggaaagaccagcaagaaggaaagagagaaagagaaagtcagagaaagagacagagagaggaagagacagagagacagaacgttaaagagggtgtcagaaacagagacaaacaaaaggagtcagaaagaaggacagacacagaaagtcaaagagagagttaaaaagagaggaagagacaaagaagtcgaagagagaaagagagagatggaagt

SEQ ID NO: 10 - DNA, 2421 bp, Homo sapiens
ctttgcagataaatatggcacactagccccacgttttctgagacattcctcaattgcttagacatattctgagcctacagcagaggaacctccagtctcagcaccatgaatcaaactgccattctgatttgctgccttatctttctgactctaagtggcattcaaggtaaggaacatcaaaggatacttaatttgtaaaatgagaaataggaataggtataaattctaaaaatacagaaataatgtatttgtaaaagtttcactgcatgcttataaataagagggaaataaatagagattccctcagatcataaaacttatatgaattgaagtgagagaaacaaatagaataagagaaagagaaggaaaaagggaaggaggacagaagagatggggaagagggaggatagagagagaaaatgtgagggaatgcggacagagatgagatacagatacttccttacctaactaagctcaatgaaccacatgaactgtgcttaagggtttgactttataatcaacaagctgcaattcttttcttccagataatcaactctttaatcatttacagttgtgttatgatgtgatccattcctcctcagattaagtgactatttgctgatatggggatataggttctgctaaataccaccagtctacattaaatgcctaaaatgaacactgtgctaaccttctctgctgttcctcttttcctacaggagtacctctctctagaactgtacgctgtacctgcatcagcattagtaatcaacctgttaatccaaggtctttagaaaaacttgaaattattcctgcaagccaattttgtccacgtgttgagatcatgtgagtgaaatcccatctgattatcacttccctggttgtaattatatactgtattaaatatgtaatgataataaaaaaagatcagtaaagggtttgtgatgattctaaaactaatgtacagcaaacaaaaacatgcagagtgaaacttaaatgtctgacttcagaactgcgtatgccatctgttttattgacccaacacagttttaaatattttcatccctatttatttctacagtgctacaatgaaaaagaagggtgagaagagatgtctgaatccagaatcgaaggccatcaagaatttactgaaagcagttagcaaggaaaggtaggtttgctgttgcctgcagaagaattgctctttaggaaacggcaatcttgggagtcagaaatacttgcattgtggtttgctgtgcaatcgctggtttaaaagtatgttaccaccacgccctcccctacctccatttatttaaatgctgaggcaccatcttgtgtgataagtatcagaagttaccctgattaccagtcaaccttgaagtacagctataactatctaagcaaaactgacaacattttccccaagtctttcatggttgaaaaaagcaacccctataatccataatgaatgcatagcagcaggaaagctcagttatctattctatgaactcggtactttccaaacacaacccaatctgaagccagagtcagactatcacacttttatatcccctttctcttcttacaggtctaaaagatctccttaaaaccagaggggagcaaaatcgatgcagtgcttccaaggatggaccacacagaggctgcctctcccatcacttccctacatggagtatatgtcaagccataattgttcttagtttgcagttacactaaaaggtgaccaatgatggtcaccaaatcagctgctactactcctgtaggaaggttaatgttcatcatcctaagctattcagtaataactctaccctggcactataatgtaagctctactgaggtgctatgttcttagtggatgttctgaccctgcttcaaatatttccctcacctttcccatcttccaagggtactaaggaatctttctgctttggggtttatcagaattctcagaatctcaaataactaaaaggtatgcaatcaaatctgctttttaaagaatgctctttacttcatggacttccactgccatcctcccaaggggcccaaattctttcagtggctacctacatacaattccaaacacatacaggaaggtagaaatatctgaaaatgtatgtgtaagtattcttatttaatgaaagactgtacaaagtagaagtcttagatgtatatatttcctatattgttttcagtgtacatggaataacatgtaattaagtactatgtatcaatgagtaacaggaaaattttaaaaatacagatagatatatgctctgcatgttacataagataaatgtgctgaatggttttcaaaataaaaatgaggtactctcctggaaatattaagaaagactatctaaatgttgaaagatcaaaaggttaataaagtaattataactaaga

SEQ ID NO: 11 - DNA, 2421 bp, Homo sapiens
agatgacttttttctatttatatttaataagatgatgaacccttcttgcattcccgaaataaacctcaactgttacagtgttttattcttttaatatgtacgaagtacatgttaagcaagttatttcctaagcagccccacaaactgggcactactaccatcctgctctgcccctccctcactctacttcagccacttcagccacaatggcctctcctcactgcccctctgatgcaccaagcttgttctcacctcaggaatgtgcaacacctgccagacttgctgttccccggagcctccatccccagatatcctcatatatcatcctcctcttcatttgtgtctctgcttacatatgacctatttacagaagcctttcctgtctaccccccatgaaatagaaatcgcattccaatcttgtctctaccccaatgctgtttcattttgtctgtagcaattgtcatcatctcatatatattcacatgtggaaaatacacaaaatgtttaacttcttttaatttacattccatttccccatgaattgaagctccatgacagcggagatttttctctgctttccctgttgctcacttcccagcaccaagagcaggcctggcacatgggaagtacttactatttattgaatggatgaatgaacaaatgaatgaatggatacttattttacacataagaaaactgaagcttatagaaattaagtaactaaaatcacacagaagcacagctgaaactaaaacctacgtctaactttcaattcctgacccttaaccattaaaacaaatgacaggtgactttaggccactgaaaatgctcatataatcttatgaattctaaagcacaagttaatcacaccattgattgaaagtctgaggaatactgtatagacaagcccctgtacaaggtaagcaaaagaatcagaggatggcctccaaagaattccctggacattatgggaattacattgttagccttcctactgatacccataagcctcacagcaagcatcatgaagctgtgaccttcatctgcacatgcccttgtatacccaaaagataaaactggatgcttcagggccgaatggccaataaacacgtgtttattactggcatgggcagacacacatactgaaagtaccatttcccagcggactagccatattatgatcagtacagacactaaagatttagctttgaaaaaactatttgctcttccaaagctgaagaatcttctgtgatttcaacaggcaagttacagtcaggtattcttaatgttcttttcctcctctctcactgggatactttctttccttcagacaacgtcaagcgaaaaacaaaatttcacaaatctccatttctgacactaaacagtacagtatctttattttttttataatttaatcaaaccctgtattttagaactgtggggctgatccaacattgcaatgtgtcacatttaattccatcaatgtaaagcataatgagcaaagattaaggtagtgaggcataactaaatgttttgaacctgtgaatttcaaaagcaaggcccatttgtgttattttctaaatagtaaataaaatcattttccaacatttcactatcaaattacagtaatttttccaccagtacacacttgaggaaagccacaaaaagacttttccaacagttcattctgttattgctcataaccttctaaatacttctcctcattggcttctattcaaaggtaaatggaaagcagtaaaatttatggaaaatatattcaactgcttaaaatacatcaaccaaaaaaaagattttagagctgtattatgagttgtgaaattgcattgccttcacttacctttcagtttcactggtaggtaacaaaactgacagactggtcaagttccaaaacatcccctatatagagcctgactcttccatctcaaattctcaccttggtcaaggccagagtaaacacctgtccttcacatttttacacaacatcactttgtatgctacaaatataagctttcataccagggaggaagcaaattccaggacactggaaacatttctgctctcttaaaccagtctgttgattgttcccttgactttctcagctgtcaggatagtgaaaggaggaaaactgcaaaactgtaaagtataacctgataagtttgccctttaagcttttcacacagagagaggtaaaataaaactcaagtctaaggtttaaaattgagctatgaatattatattctagcactagacaaaaatgttgcaagattttaataaaataagattattaaaatcaatttttacatttcatgggccaaggagagacatcaaagaatgtttaactaacattttaaagatactatactttataaagttaagaagaaaaatgacaactgcaccagt

SEQ ID NO: 12 - DNA, 1227 bp, Homo sapiens
ctttgcagataaatatggcacactagccccacgttttctgagacattcctcaattgcttagacatattctgagcctacagcagaggaacctccagtctcagcaccatgaatcaaactgccattctgatttgctgccttatctttctgactctaagtggcattcaaggagtacctctctctagaactgtacgctgtacctgcatcagcattagtaatcaacctgttaatccaaggtctttagaaaaacttgaaattattcctgcaagccaattttgtccacgtgttgagatcattgctacaatgaaaaagaagggtgagaagagatgtctgaatccagaatcgaaggccatcaagaatttactgaaagcagttagcaaggaaaggtctaaaagatctccttaaaaccagaggggagcaaaatcgatgcagtgcttccaaggatggaccacacagaggctgcctctcccatcacttccctacatggagtatatgtcaagccataattgttcttagtttgcagttacactaaaaggtgaccaatgatggtcaccaaatcagctgctactactcctgtaggaaggttaatgttcatcatcctaagctattcagtaataactctaccctggcactataatgtaagctctactgaggtgctatgttcttagtggatgttctgaccctgcttcaaatatttccctcacctttcccatcttccaagggtactaaggaatctttctgctttggggtttatcagaattctcagaatctcaaataactaaaaggtatgcaatcaaatctgctttttaaagaatgctctttacttcatggacttccactgccatcctcccaaggggcccaaattctttcagtggctacctacatacaattccaaacacatacaggaaggtagaaatatctgaaaatgtatgtgtaagtattcttatttaatgaaagactgtacaaagtagaagtcttagatgtatatatttcctatattgttttcagtgtacatggaataacatgtaattaagtactatgtatcaatgagtaacaggaaaattttaaaaatacagatagatatatgctctgcatgttacataagataaatgtgctgaatggttttcaaaataaaaatgaggtactctcctggaaatattaagaaagactatctaaatgttgaaagatcaaaaggttaataaagtaattataactaagaaaaaaaaaaaa

SEQ ID NO: 13 - protein, 98 aa, Homo sapiens
MNQTAILICCLIFLTLSGIQGVPLSRTVRCTCISISNQPVNPRSLEKLEIIPASQFCPRVEIIATMKKKGEKRCLNPESKAIKNLLKAVSKERSKRSP

SEQ ID NO: 14 - DNA, 2301 bp, Homo sapiens
aaggcaagagatctaggacttctagcccctgaactttcagccgaatacatcttttccaaaggagtgaattcaggcccttgtatcactggcagcaggacgtgaccatggagaagctgttgtgtttcttggtcttgaccagcctctctcatgcttttggccagacaggtaagggccaccccaggctatgggagagatttgatctgaggtatgggggtggggtctaagactgcatgaacagtctcaaaaaaaaaaaaaaaagactgtatgaacagaacagtggagcatccttcatggtgtgtgtgtgtgtgtgtgtgtgtgtgtgtgtgtgtgtggtgtgtaactggagaaggggtcagtctgtttctcaatcttaaattctatacgtaagtgaggggatagatctgtgtgatctgagaaacctctcacatttgcttgtttttctggctcacagacatgtcgaggaaggcttttgtgtttcccaaagagtcggatacttcctatgtatccctcaaagcaccgttaacgaagcctctcaaagccttcactgtgtgcctccacttctacacggaactgtcctcgacccgtgggtacagtattttctcgtatgccaccaagagacaagacaatgagattctcatattttggtctaaggatataggatacagttttacagtgggtgggtctgaaatattattcgaggttcctgaagtcacagtagctccagtacacatttgtacaagctgggagtccgcctcagggatcgtggagttctgggtagatgggaagcccagggtgaggaagagtctgaagaagggatacactgtgggggcagaagcaagcatcatcttggggcaggagcaggattccttcggtgggaactttgaaggaagccagtccctggtgggagacattggaaatgtgaacatgtgggactttgtgctgtcaccagatgagattaacaccatctatcttggcgggcccttcagtcctaatgtcctgaactggcgggcactgaagtatgaagtgcaaggcgaagtgttcaccaaaccccagctgtggccctgaggcccagctgtgggtcctgaaggtacctcccggttttttacaccgcatgggccccacgtctctgtctctggtacctcccgcttttttacactgcatggttcccacgtctctgtctctgggcctttgttcccctatatgcattgcaggcctgctccaccctcctcagcgcctgagaatggaggtaaagtgtctggtctgggagctcgttaactatgctgggaaacggtccaaaagaatcagaatttgaggtgttttgttttcatttttatttcaagttggacagatcttggagataatttcttacctcacatagatgagaaaactaacacccagaaaggagaaatgatgttataaaaaactcataaggcaagagctgagaaggaagcgctgatcttctatttaattccccacccatgacccccagaaagcaggagggcattgcccacattcacagggctcttcagtctcagaatcaggacactggccaggtgtctggtttgggtccagagtgctcatcatcatgtcatagaactgctgggcccaggtctcctgaaatgggaagcccagcaataccacgcagtccctccactttctcaaagcacactggaaaggccattagaattgccccagcagagcagatctgctttttttccagagcaaaatgaagcactaggtataaatatgttgttactgccaagaacttaaatgactggtttttgtttgcttgcagtgctttcttaattttatggctcttctgggaaactcctccccttttccacacgaaccttgtggggctgtgaattctttcttcatccccgcattcccaatatacccaggccacaagagtggacgtgaaccacagggtgtcctgtcagaggagcccatctcccatctccccagctccctatctggaggatagttggatagttacgtgttcctagcaggaccaactacagtcttcccaaggattgagttatggactttgggagtgagacatcttcttgctgctggatttccaagctgagaggacgtgaacctgggaccaccagtagccatcttgtttgccacatggagagagactgtgaggacagaagccaaactggaagtggaggagccaagggattgacaaacaacagagccttgaccacgtggagtctctgaatcagccttgtctggaaccagatctacacctggactgcccaggtctataagccaataaagcccctgtttacttga

SEQ ID NO: 15 - DNA, 2301 bp, Homo sapiens
aggaattgaactcagctctgccccaagcggacctaatagacatctacagaactctccaccccaaatcaacagaatatacatttttttcagcaccacaccacacctattccaaaattgatcacatagttggcagtaaagctctcctcagcaaatgtaaaggaacagaaattataacaaactatctctcagaccacagtgcaatcaaattagaactcagaattaagaatctcactcaaaaccgcacaactacatggaaactgaacaacctgcttctgaatgactactgggtacataatgaaatgaaggcagaaataaagatgttctttgaaatgaacaagaacaaacacacaacataccagaatctctgggacgcattcaaagcagtgtgtagagggaaatttatagcactaaatgcccacaagagaaagcaggaaacatccaaaattgacatcctaacatcacagttaaaagaactagaaaagcaagagcaaacacattcaaaagctagcagaaggcaagagataactaaaatcagagcagaactgaaggaaatagagacacaaaaacccttcaaaaaattaatgaatccaggagctggttttttgaaaggatcaacaaaatagatagaccactagcaagactaataaagaaaaaaagagagaagaatcaaatagacacaataaaaaaatgataaaggggatatcaccaccgatcccacggaaatacaaactaccatcagagaatactacaaacacctctacgcaaataaactagaaaatcaagaagaaatggataaattcctcgacacatacactctcccaagactaaaccaggaagaagttgaatctctgaatagaccaataacaggatatgaaattgtggcaataatcaataccttaccaacaaaaaagagtccaggaccagatggattcacagccgaattctaccagaggtacaaggaggaactggtaccattccttctgaaactattccaatcaatagaaaaagagggaatcctccctaactcattttatgaggccagcatcattctgataccaaagccgggcagagacacaaccaaaaaagagaattttagaccaatcaatatccttgatgaacattgatgcaaaaatcctcaataaaatactgccaaaccaaatccagcagcacatcaaaaagcttatccaccatgatcaagtgggcttcatccctgggatgcaaggctggttcaatatacgcaaatcaataaatgtaatccagcatataaacagagccaaagacaaaaaccacatgattatctcaatagatgcagaaaagacctttgacaaaattcaacaacccttcatgctcaaaactctcaataaattaggtattgatgggacgtatttcaaaataataagagctatctatgacaaacccacagccaatatcatactgaatgggcaaaaactggaagtattcactttgaaaactggcacaagacagggatgccctctctcaccactcctattcaacatagtgttggaagttctggccagggcaattaggcaggagaaggaaataaagggtattcaattaggaaaagaggaagtcaaattgtccctgtttgcagacgacatgattgtatatctagaaaaccccattgtctcagcccaaaatctccttaagcagataagcaacttcagcaaaatctcaggatacaaaatcaatgtacaaaaatcacaagcattcttatacaccaacaacagacaaacagagagccaaatcatgagtgaaatcccattcacaattgctttaaagagaataaaatacctaggaatccaacttacaagggatgtgaaggacctcttcaaggagaactacaaaccactgctcaatgaaataaaagaggataaaaacaaatggaagaacattccatgctcatgggtaggaagaatcaatatcatgaaaatggccatactgcccaaggtaatttacagattcaatgccatccccatcaagctaccaatgcctttcttcacagaattggaaaaaactatttttagttcatatggaaccaaaaaagagcccgcattgccaagtcaatcctaagccaaaagaacaaagctggaggcatcacactacctgacttcaaactatactacaaggctacagtaaccaaaacagcatggtactggaaccaaaacagagatatagatcaatggaacagaacagagccctcaaaattaatgccacatatctacaactatctgatctttgacaaacctgagaaaaaccagcaatggggaaaggattccccat

SEQ ID NO: 16 - DNA, 2024 bp, Homo sapiens
aaggcaagagatctaggacttctagcccctgaactttcagccgaatacatcttttccaaaggagtgaattcaggcccttgtatcactggcagcaggacgtgaccatggagaagctgttgtgtttcttggtcttgaccagcctctctcatgcttttggccagacagacatgtcgaggaaggcttttgtgtttcccaaagagtcggatacttcctatgtatccctcaaagcaccgttaacgaagcctctcaaagccttcactgtgtgcctccacttctacacggaactgtcctcgacccgtgggtacagtattttctcgtatgccaccaagagacaagacaatgagattctcatattttggtctaaggatataggatacagttttacagtgggtgggtctgaaatattattcgaggttcctgaagtcacagtagctccagtacacatttgtacaagctgggagtccgcctcagggatcgtggagttctgggtagatgggaagcccagggtgaggaagagtctgaagaagggatacactgtgggggcagaagcaagcatcatcttggggcaggagcaggattccttcggtgggaactttgaaggaagccagtccctggtgggagacattggaaatgtgaacatgtgggactttgtgctgtcaccagatgagattaacaccatctatcttggcgggcccttcagtcctaatgtcctgaactggcgggcactgaagtatgaagtgcaaggcgaagtgttcaccaaaccccagctgtggccctgaggcccagctgtgggtcctgaaggtacctcccggttttttacaccgcatgggccccacgtctctgtctctggtacctcccgcttttttacactgcatggttcccacgtctctgtctctgggcctttgttcccctatatgcattgcaggcctgctccaccctcctcagcgcctgagaatggaggtaaagtgtctggtctgggagctcgttaactatgctgggaaacggtccaaaagaatcagaatttgaggtgttttgttttcatttttatttcaagttggacagatcttggagataatttcttacctcacatagatgagaaaactaacacccagaaaggagaaatgatgttataaaaaactcataaggcaagagctgagaaggaagcgctgatcttctatttaattccccacccatgacccccagaaagcaggagggcattgcccacattcacagggctcttcagtctcagaatcaggacactggccaggtgtctggtttgggtccagagtgctcatcatcatgtcatagaactgctgggcccaggtctcctgaaatgggaagcccagcaataccacgcagtccctccactttctcaaagcacactggaaaggccattagaattgccccagcagagcagatctgctttttttccagagcaaaatgaagcactaggtataaatatgttgttactgccaagaacttaaatgactggtttttgtttgcttgcagtgctttcttaattttatggctcttctgggaaactcctccccttttccacacgaaccttgtggggctgtgaattctttcttcatccccgcattcccaatatacccaggccacaagagtggacgtgaaccacagggtgtcctgtcagaggagcccatctcccatctccccagctccctatctggaggatagttggatagttacgtgttcctagcaggaccaactacagtcttcccaaggattgagttatggactttgggagtgagacatcttcttgctgctggatttccaagctgagaggacgtgaacctgggaccaccagtagccatcttgtttgccacatggagagagactgtgaggacagaagccaaactggaagtggaggagccaagggattgacaaacaacagagccttgaccacgtggagtctctgaatcagccttgtctggaaccagatctacacctggactgcccaggtctataagccaataaagcccctgtttacttgaaaaaaaaaa

SEQ ID NO: 17 - protein, 224 aa, Homo sapiens
MEKLLCFLVLTSLSHAFGQTDMSRKAFVFPKESDTSYVSLKAPLTKPLKAFTVCLHFYTELSSTRGYSIFSYATKRQDNEILIFWSKDIGYSFTVGGSEILFEVPEVTVAPVHICTSWESASGIVEFWVDGKPRVRKSLKKGYTVGAEASIILGQEQDSFGGNFEGSQSLVGDIGNVNMWDFVLSPDEINTIYLGGPFSPNVLNWRALKYEVQGEVFTKPQLWP

SEQ ID NO: 18 - DNA, 26803 bp, Homo sapiens
cttgctctgtcacccaggctggagtgcagtgctgtgatcatggttcactgcagccttgaactcctgggctctggcaatcctcctgcctgagccttctgagtagctgagactatagatatgggccaccacacctggctaatttttaattttttttagtagagatgaagtcttgctatgttgaccaggcttgtgggagttcagtcaggctggtggaaaaaattttaaagatagttataagaaatagacacaaaccttcttgtaaggctggagagggtttacattgcttcagtaacagatttggctgaaagcagcctaatcctctctacctttagctgatagcaaaaatgaaaataacaagggaatgtgaggaagtttatctaaatagcttgcttactcatgtggtcctaaaaccaaactttgatcaacctcaggtgcataattgctctctactcagggggtgagcaatgttaattaccctctagtggtgtttactcgagacctttgtcatttaatctgtattaaataaatgtgaactttgctagcttattgaggtgatgctccagatgcagagcagagccccttagccagactgacaggcaaaatatctgtgtcagtgtatgtctctcatccatcactggttcagggtctgcgggctggattcctgcacaggctggtcttgaactcctgggctcaagcaatcctcccgcctgagccttctgagtagctgagactacagatatgggccaccacacctggctatttttaacattttttagtagagatgaagtcttgctgtgttgcccaggctggtcttaaactcctgggctcaagagctcctcctgccttggcctcccaaagtgctgggagtacaggcatgagtcatggtgcccagacggacatttttttaaaaataaaggaatactcctgaaacgctgaagtcttctttgtacccctctgtgataacatgaatagcctcttaatgacaccaaggagcaagacaagttagtcccaaagtagctcacatagatgatgataaaggaatgaggggtgggtgtgatctatgcaaaaaacccttactctttaatgggttgctgtttctaacataattgcaacagtaccctacattgctataatgcattatagttttcaaagtgcttttgtggcctccataatagagaggttgtgaggtaagcttcaaccacggctgccctactacccaagagtggacacacaatgatgaataggtcaatttctgcctcttagtttcttagctagggaggggcacttactggaacagcacagaaaacagagtctttggcccagttggagaatctttatcaggttatgctacttcaagctttcctcctgttaaatgtgagaggaataaatccctgttccttggatcagtgtgactctgaaacagctggaggagagacagctttaggcaggttgaaacagagagctccagcatatgtactttttttttttttttgagatggagtctcgctctgtctcccaggctggagtgcagtggctcgatcttggctcactgcaagctctgcctcccaggttcatgccattctcccgcctcagcctccctagtagctgggactacaggctcccgccaccacgcccggctaatttttttgtatttttagtagagacagggtttcaccatgttggccaggccagtcttgaactcctgacctgaggtgatccacctgcctcagtctcccaaagtgctgggattacaggcgtgagccactgaacttggccaagtgcactacttttaaaagttaaagtattatgcagccatgagggaatattgtgcaagaagaaagcttttacaagaaaaacttgaaacattggtatttttgcctcctttttaacaactagagtcgttttgggagttgtttcttgtcgaagaaacaacccatgtttattttcccagtatggcaggaccatgtaggaaagcaaaattacccctcaggagaggaaattctctgacactctataaggctccataaccctcctctgaactgtggccaacaagattgggtagcactttttaaggtagtttaagaaaaataggctgtgcatggtggtttatgcctgtaatcccagcactttgggaggccgaggtgagtggatcacctgaggtcaggagtttgagaccagcctgaccaatatggtgaaaccccatctctactgaaaatacaaaaattagccgggtgtggtggcgggcacctgtagtcccagctactcgggaggctgaggcaggagaattgcttgaacctgggaggcggaggttgcagtgagccgagactgtgccactgcactccagcctgggtgacagagcaggactccatctcaaaaaaaaaaaaaaaaaaaagaaagaaagaaaaatatatagtgagcccaataaagctgtataatctaaatcaaacatgacttgcatgcctggagactttgcactagaaaaatatttctacctaaaaaatcaaattttattttctttctcacaaatattcaatctgctttcatctcagttcttcctaccttgtcaaacctctccccacatttcctattctttttctctccagcctgatatctctcattatactgcttaagagaaatgttatgttactattcttttctcccagaactgtttctctggttctttaaggtgtctgagtacacactgtgccttcttccttttagccctctcttctccttgttccctgagccttacctttatgaccttagaacttcaagttcccactacaattttaaatatagactattttgcttttcctcctactagggagcttaaattgcctctaattacactgttttcccgagtccttcctctcctttgcaatttagatatagcacagaagcacattttgcttgactgtcctctgaactgtcatgctgttttgatgtggttctattgtccaagagtcttggttaaataatagcccagcatcccacctgtgtttaaaagaactgcttcacaggcaaatcaaaaagcccatggatccgaagtcacaatgggcgttgctattcaaacagcaccagattgctattcaacgcttggttgaaaaataaatttcagtttcattcacctaatatatttccttctattttgtaggatggtatgctcttacttcaatttggacttgttcacaattgaacgttaacatagccttatagattagcctgttttcattggtccagagtattctccaaataaagcagggtctgtgcattttaagcaactcccctgaacaatttcatgggcattctcaaatttgagaactacctgaaaagctgtgttggagaaaagaacaaccaatgaatgtggcaggacagaatattgaacattaacttcccttttcctcttctcccatctgttctcttccattatccctacccgtccgctcagtctcgttattcaggcaacagttattttgccattatttcctcaagaaaggaacaaaagtaaacacaattgctttctgattttttttttttttttgcattttaaaatggactttgaaaccataagcaaagaggtgtttaagagtctttccaaagccaaaaatgaaggttttgaaatttcaaagtcactgccttgaagagactcgaggtttggagtgtgtacagtatgtcggagctggacttttctccttcctgagactagataacggtctgaatccaagacagttttcatgatttcagaggaagtggtcaagtggtctgtgaggtagaccttctgcttaagagcagtcaggaggccgggtgccgtggctcacgcctgtaatcccagcactttgggagaccgaggtgggcggatcacctgaggtcaggagttcaagacaagcctgaccaacatgcagaaaccctgtctctactaaaaatacaaaaaattggccgggcacggtggcacatgcactccagcctgggcaacaatagtgaaactccatctcaaaaaaaaaacaaaaaaaagagaagaaaagaaaagaaaaggagcagtcaggatgtgtgcctccaaagctgaggtagacaaaaagataccagagttctagaggcctgccaggcacagcagcagcagcagaaggaaggtgtgggcgagaacagggcagccaggcgtgtgccacctcccagacacaattattgggaatggagggcaagtggtgatgggagaaaatcttgacttaattgatgtcaagattaaagaaatgccacctggtggcatttaagttcacacataggtaaagaaagttatgcatttactgtgaaagtcatcccactatttagtagaaacaggagatctggattctggtcaagagtctcttttgccaactgtggcaccactgagcagcggcacagcttttgtgaatcctgggttcttcattattaaaatggggacattagcgttgggttgagtataagaaatggacatttttgcaggtcaaaaatggttgaatatttgcattttcatatgattcaaccgaatacttacttcacaggcataaggaaaaaaatagaataacatactaacaactgtccctggagtaagtacttaacaaatacatgatttataaagaagatatgtgaaagatatttgtaagtacatgatttatagaaagatatgaaagtatgtaaacccttgtggtctaatggtcacagaataatctgagcttaatatccctgctccctaccatacagaaggcaaaatgcctattaggggttttctttcttcaccctctccttctttttcctcctcctcttgactcctcctcatcctcctctttcttcttccccttattaatgtctaaaaaggggctgagcatggtggctcatgcctgtaatcctagcactctgggaagctgcggcaggtggatcacctgaggccaggagtttgaaaccagcctggtcaacatggcaaaaccccatccctactaaaaatacaaaaattacccaggtgtggtggcaggcacctgtaattccaactacccgggaggctgaggcaggagaatcgcttaaacccgggaggcagaggttgcagtgagccaagattgtgccactgttgtccatcctgggtgacagagggagactctgtctcaagataaataataataataataataatttctaaaaaggtaatacattttcatagttcaaaaaccaaaaggtataaaaggaaatacagtaaaaaatttcctatcatatcactgtctagagtactattccttatatattttcctgatttttgagtattttaaaatgtgagtgttggatatgagtgttggatttaaaaagttttatgataatttgtgtatatttgtgtgtgtgtgtgtgtgtgtgtgtgtgtatagtagtccaagactatcagtttatgaataataagaggagacccatggaaaaccagtccctttgaccaagttcactcagataatcagcagcagggcttggacattaattacagttatccaacatcctttgaggtctcacatgacaaattacaaatatggagtgtaaatgtaacccactttgctaggcaaaaaaagccctgtttttttaaaaaatatatatttttggcttatgggcaacagaagccagggagacgtacagtcaaacctcatttctcatggctttcatatctgcaaattctcctactcattaaaagttatttataactcccgaatcaatacccacagcacttttgtgatcattggcagacatgtgcagaaaagaaaaaaaaattgagttgttgattgcacacattcccagctgaatttcaacaaagcaacactctgccttcccacttcagctttcttactatatgtgtgtcctttttctgtttatttagtaccatgtttttcacactttcgttctttttggtggtgattttgctgtttaaaatggccaacaagtgtagtgctaagtgctgcgtagggttcttaagcacaagaaggctatgatgtgccttatggagaaaatacgtgtgttggatcagtttcactcaagcatgagttatggcgctattagctgtgagttcaatgttaacaaatcaacaatatatgctaaagtgtctttaaacagaaacacacataaaacaaggttatatgtttggttggcaaaaatgttataaccagaagcttgcagaaacctaaccctgtatttcccttaagagcaatggttcattattcactaattcaatgtttacagcaactttataaactataactaccatgaataatgagaattgactatgttttagatcataatacctgaagtgaagttttccatcatggtttttagttcttagagtccatttaagttttttaaaaatatgatagctatcctatcacatcccacattcttgagattaaaaaattaatcttttatttggtacagaaaaggctcctgcgtgcatttttggaggggctggaccgctgaggaagtcatggttggctcaagtggtttaaatgcattgctaatttcatagcctctgaaccacttatgaaacaatactgatgatatgtcagtagctatgtttgcagctccttcaggaatgcttatatcttttactgctggtaaagaagaaatttatagtaatagattttttttttttttagatagagtctcactctgtcgcctaggctggattacagcggcttgatcacggtttactgcagcctggatctcccaggctctcctactgtagcctccccagtaactagggcccccacacaggcatcaccacacccagctcatttttttatgttttatagagacagggtcttactatgttttccaggctggtctcaaacttctgggctcaagcaatcctcctactttggcctcccaaagtgctgaaattacaggcatgaaccactgcacctggtttatggtcatcttaagtagagacttatgagtgcgtatcattgtatcaccaatctgagactcaattttatctttctgttaatagacaatgcagtttttctgttaattacaatgaaaatcaagggttgcttagcaagtttttactcataactccaagttttgtgacttatagtgagaaatgggtataattctttgtgatttgttaaaatgcagtatttcgaggagggataacatataaaatttaacagtttcctatcattatttttatccttttgaaccactgtatactacagatagacaaaggcagctttggccacttactcctcagtgtgactaagttgaccagatgttttccagaccacaggttctgtcaagagacagtgtggagagaaatgggtaggcaggtatggaaagaagagtcagaaacagatagtgagctaatctctacaaatggctcgttatggcctgagctgtgttctcctccccgcaaaaagatatgttggagtcgtaatccccagtacctcagaatgtggccttatttggagattcgatatttacagaggtaagcaagttaaaatgagatcactatagtgggtcctaattcaatacgactggtatccttacaaaaaaggggaaatttaaccacagatacagacacacacatagggagagtgctagtgaaggtgaagtcagagattggaatgatgtagcagaagcctaggaatgccaaagattgccagcaaaccaccagaagctgggagagccacatggaacagattctccttcacagtcccctgaaagaaccaactctcctgacacctcgatttcagacttctagcctccagagctggggtcaatgagcttctctcattaagccatcatccagtgtatggtactttgttacagcagtcttagcaaatgcatggttcctcactggaaccatgaatttccatgcatttatttcatttaaataataaaacggatcccctttgtggcttgtagttctgttccatttcaaaaatccagaaaaaagatttgttcagaagctagaaatgatgaactggatcttgcccaaggtcataaaaccacaaaaccctttacagagcacaaaagtctgatttttcaaagcttctctcaaaagatgggtcactccttagtcatttaggccactgacaactgccctggactctttatttatttatttatttatttatttatttaatttttttgagacagagtcttgctttgtcgcccaggctggagtgcagtggcgtgatctgagctcactgcaagccctgcctcccgggttgacgccattctcctgcctcagcctcccaagtagctgggactacaggcacccgccaccacgcccggctaattttttgtattttgtttagtagagacagggtttcaccatgttagccaggatggtctcgaggtcctgaccttgtgatccacccgccttggcctcccaaagtgctgggattacaggcgtgagccactgcgcctggcctggactcttacatataataagcttgacttatcgtacaacttataattgatgctttcacgtcatgggaagatcaaattaatgcagagagcgactacgtttctggtgggagagcagcaggggtcttgagaggaacagcagtgttgactgtttcgctacctactctgggtgctgattacatctttctttcgtgcaggcaaatccacttggagctattttgggctcactgtgggcatcattctttgtatactctgctcctttcccccatagtttctctattgatgggggattactaaagaatgaagaaaagaacaaaatgaaagtggcttttgaaaaattttaaatgactgtcactatgtaacatattcattatttcatgtctccactggacattttggagatgtgagccttgcaatacctacatgaatgcttctatgattatgattattgttttgctcttcgcctaacaacttgccaagtattgtcaacctcagtgtgtgagatggggtccactcaaacatcagggccgaagtcaggtagttcagttaagtgaatttgataccaggaactagttacaaaggagttggaagggctggaaagccaaactggagaagaaggggaaccccagagtaacaatagcaggaagcctctaccgtctacctctagaactggggaggagctgagttaacagagtcctggagccattgctggggaagaagaaccccaactgcagaggaaaagtggccattgtgaagaaggtgatggtggagaagtcgtctgaatcaaaggggagaggatatgttggctcctttatctttttatctttcattgtcctaattccttctgggcatggttaaatgagcccaggaaatgcagttggcaggaatcagcttcctgtgacatagacagagtaagagaaggacaaaaataatgaatctgagagcaagcaggcaaatgaccagcacattaagcctagcacacagtatgttatacgggatttggggtagcaaaagatgaaggcaggtcagagaagccacaactaggggatgggcaaggtcaatgaggtatgacgggtattgtatacaggaagagggtcataaacaggagtggagtcaatacaggagactaacatatacacatcataaatattagtagagaagcataaaatagtctcctggagatcagggaaacaggaaattataggttttcaggataattcagccatatccaggaaacacacacagtgaagtaacaaagagtcaataggcttagagtggtacaattcattatgcacatgtaggaattcattccaaataataggctgaaatgtagacatgagaatccaaaaaagatgttttcttagtttttgccaatatcttagctacgttttttttggttcaacaaagtaagttaacagtcatatctgcttggaaattgtatttaggccaggtgcagtgtctcacgcctgtaatcccagcacttggggtggctgaggcaggaggatcccttgagcccaggagttagaggctgcagtgagcgacaactacaccactgcattccagtctgggtgacagaacaaaaacttattaaaaaaagaaaaaaaaaaggtcgggcgcggtggctcacgcctgtaatcccagcactttgggaggtcgaggtgggcggatcacgagtcaagagatggagaccatcttggtcaacatggtgaaaccccatctctactaaaaatacaaaaattagctgggcatggtggcatgcacctgtagtcccacctattcaggaggctgaggcaggagaatcgcttgaacccgggaagcggaggttgcagtgagctgagattgcaccactgcactccatcctgtcgagactctgtctcaaaaagaaaaaaaaggaaaagaaactattgaaatagctgatattagtttgcttacttgtcgttactctttttcatgatggattataaagaaaagttataactatttgaattttctgctgatttgaagtctctataaacagtacattcctttttggtacacagagggcacttatctgcaagaaaggcaaagaaaatggaaaagttaatgaaagaggaatcatccaatccacgaacagaatgaaaccacatacacagtgaagaaacttgtcttacattttcttccttatattacttatcattcatggtagtgactactttggggcttgagtaaagcttctctaatttattccatgtagcatcatatgtgaaaaagacaaatagatactttagacatgataataacactttattttttatttatttgtttattttgagacagagttttgctcttgttgcccaggctggagtgcaatggtgcaatctcagctcactgcaacctctgcctcctgggttcaagcgactctcctgactcagcctcccaagtagctgggattacaggcacgcatcaccacgcccagctaattttttgtaattttagtagagacagggtttctccgtgttggccgggctggcctcaaactcctgacctcaggtgatccacccaccttggtctcccgaagtgctgggattataggtgtgagccaccatgcctggcccataacaccttatttaaaaataatctgtctggatccatacaacttgtctggataactaaattggaaattattccttgttttaaagtaattcaattgaaaatttttaaatttttttgttaatcaagcactttttggtggaatctaaattaacacatgtaggagatgcctgtttcactaattacacaggcatcttgcagtaattaatgtctgggaggaaggaatgtcttttgcttactctcttcttcttcacaaaaatgtgaattttggaaagcaataatggaagcatgtagaattatagaaatacaaatgtatataactatcacaaaaaaatgaggccaaaggactattcagatataattaggctatggtagctgtaattatctaggaaattaataaaattcattcacctagaaattattagtgagcatcaaatatgtgtcagcactaggctagggtctcagaacgtacagataaatcatagttctggcttcagggagttatatagattagagataaaacctaactacaggggctgggcacggtagctcatacctgtaatcccaccactttgggaggccgaggcgggtggatcgcctgaggtcaaggagtttgagaccagcctggccaacatgataaaatcctgtcactactaaaaatacaaaagttagccgggaggtagtatgtgcacctgtaatcccagctactcgggaggctgaggcaggagaatctcttgagcctgcggtggaggttgtggtgagctgagatcacgacactgcactccaatctgggcgagagagtgagaccctatctcaaaaccccaaacaaaacaaacaaaaaaaccaaacctaactacagggctatgagagatgactactggcaaggagccacaggtagaacaaaggggatgtgtccccaggcaaagggtagtcagcaagcctgcaacctcagggttcccggatctgagcctctggctcttggctaggcaggccccaagcgttggcctcctgccatggcaagctccagcctggtctcccaccttgagctaacattcatatgttgtagacacagccacgcttcctgcttacctgtcacttccagttctcgaaggcacccttttcaaatgaaaatccgccccttttcacatcaaacagctcatctggtcctgtggattacatttctcagaaatgcctctgaacattcgcctcctctccacccccactgcctctgctacagtgcaggtgctcgccatttctgatttgttctgtcacacactcgtttatcaggtctctccatctcctgttttgacatgctgtaaagcaatttgccactggaaaaaagggctctctttttttttttgagacggagtctcgctctgctgcccaggctggagtgcaatggcatgatctcggctcactgcaacctctgcctcccaagttcaagtgattctcctgcctcagcctccctaaagtctgggattacaggtgcacgccaccaagcccggctaatttttgtatttttagtagacgtggggtttcaccatattggccaagctggtctcgaactcctgacctcaggtgatccacccgcctcggcctcccaaagtgctgggatttcaggtgtgaggcatcgtgcccggcctctctttccaaagtatgttattatttttcccaagaccctttgacggatcctcatttcctacacacagtggttctcaaacttggatgtactccagaattacataggaaattcttcatttttttagacgaggtcttgctatgtttctcaggttggtctcaaactcttgacctcgtgtgatcctccggccgcagtctcccaagtagctgagattataggcgtgccactgagcccagctggaaatttttttaaaacacagattcctctgaatcaaaatttctagaagtgaggtctgagcaatctgtatttttaacaagttatccagatggctctttactgtcagtctggttccagctgagggagttttagaattacaaggcaaagtccaaacttagcacacaaagtcattcacatcaactcttcccctgtacacaccctatgtcatagccagagttgtaacccatttcttaaacacccagggttcttttaagtctctgtgtcattgtatgttattttctctagaattgcctttaacctcctttccaccctggaaagcattccctaagccatctttgaagctttctttgatctctaacttagagtcctcctctccttctaaagccctgtgttaatcacttgtcatggtgtactttaatttttacttgcctgtttctctttacggtactttgacttcaaagggtggggctgcaaattagtcatctccttagagtccagccttgttcctagttcctaactggcacttaatataaacgaatgaatgaatggacaaatgaagagaatgctagttatgataaagaattggccgtgtatgagactacttctctttatgaactaaataattatatgcctttcaataaaatactagtacacgtagctagcacaagctcatcagcatttgagatgatatggaaaccaaaataaacaaatgctaccacaaaaacataatgactgctttccccagtgcaggactgatggaatcatcaaacattgagattaatgtaatgtttggcagatgtccagtgtttttatttttcatttgcctttgtgttcatttatggactaacaatataataaacacacacatactcacagtacatcttttttttttttttttttgcaaagcccagttttcttcatcgcatatctttgttttcttcaagtatccccttacttaatgttggtagtattttttttaatgaaatataaatccctaaccaccaagcaagaaatgagactcttaattgcatcagtttacagtgcaatgtgagtgtaaatagtgtaaattgaatttttaatggacttttttttttcccgtttttgcttgccttacattcattatccctccctgggtaataaacatttatttttccctttgtaaccactcctccccttctgtccatgtggttctttttagtggagctggtggtagggatgtggcatgagattcaagcttggccacctggagtcactgtgttgtgctccagaaggacacctgatccaagtcagccagtaagagtgagccccaggatttttgcttggaccactgaggaaaagtgtactctgccctgtggctgatcaaccattaggatataagccattgttgtagctgtgtgagtcaagctacctgagaatgaggacaacacagtggcaagcaacaccaagagagaaaaagaggcagattctgatgacatttttgagcctttgcatccagctatgcctgaatccaatttatcccctggaatttacacttacttgagctccacccacttgaaagaaaacatttctttttattcttagcctgatttgaatttggcctctctcatttactacccaaagtgtcttgaccactagaatattatgccagactttacagcatcattgaatttgccactttccagaagagttgtgtgaattttcaatgtagcttttaccttctatgagtatctagagatatatttaagtagaagtactccactagtttgttgtgagatcttaagtcacttaatttctctgtaccctagttccctcatttgctagacctagggagctataatgttccttctgcaaaattcttattttgtgaaatattctagaatgtctaactgatacactgctagaacaactgactgctatttaagaagagttgactgctatttaaggatcataattctctaggcataagtgctgtgacggcacagcgtgtgcatcggggctgaggggtggggtggagcagaaagtaggaggagaaagtttgataaacttccttttggataaattgaaaacagtcaaataatttataatttcttatattatcattattagcttcttctataattaggagacttgttccaaaatgtgagaattgtcacaagttgtcaaattcatcaaaggaagaaaatggatgtctcacaaaaaagtatgctcagtccaatttcttctcgtcacactggaacaaactgaacagttttacacagagatgagaagcctggacatttttcaaatatgttttgaagagaatggcaatgcctgagacagaagtaggaaaaagcaatgaatatttaaaaatctgagctggtgtaaaactagaaatagttttagtaagaacaatgtgatgtgctacactaagtgaaatgtatacattgggccacattataatcaaaaataagaatgtacttttattcatcttttatttaaacaataatcaaggtggcgggcgcggtggctcatgcctgtaatcccagcactttgggaggccaaggtgggtggatcatgaggtcaggagttcaagaccagcctggacaacgtggtgaaaccccgtctctactaaaaatacaaaaattagctgggtggggtggcatatgcctgtaataccagctgctcggggggctgaggcaggagaatcgcttgaacttgggaagtggaggttgcagtcagccaagattgtgccattgcgctccagcctgggtgacagagcaagagactctgtctcaaaaggaaaaaagaaaaaaaaaaaatcaaggtaccatttgtaccatttcctggaatttctccaaagtggcaaggtcacatgtttatacattagactcccagtttaacacacagcagacaataactttttttttttttttttgagatggagtctcgctctgtcacccaggctggagtgcagtggcacaatcttggctgactgcaacctccgcttcccgagttcaagcgattctcctgcctcagcctcccgagtagctgggattacaggcatatgccaccatgcccagctaatttttgtatttttagtggagatggggtttcaccacattgtccaggctggtctcaaactcctgacctcataatccagccacctcagcctcccgaagtgctggtccacccttccttcttttctcccttccatccttctcccttttattccatttttctaaatattagaccatagtacaaatcaaaagtcacaaactgataggctgcaatgtagatacagctgggaaaatgttttgtttgcagaacactggggaaatttaacatgaaaaactggaagatctcaatccacatggccacatggtaatattattaatgttgcaggggctttccaattcaacatgtcctctgcatccctactatttatactgccactcatccacctttctgtattactggcctatcacctatacacgtttgagtttatattcttctggctttacttagcaacttaccttttatatttaacattacaacatggtattatcaattagtattcgattcagttgcatataaccaaaaatgccaaattatactggcttaaacactaaggatttatttttctgtcatataaaacaagtctggaggtgggtagtccagggctaatatgacactccagtgtcacaaggtacctgggctccttctatttatcttttttttttttttttttgagacggagtcttgctctgtagcccaggctggagtgcagtggtgcgatctgggctcactgcaagcttcgcctcccgggttcacaccattctcctgcctcagcctccggagtagctgggactacaggcgcccgccaccacgcccggctaatttttttgttatttttaatagagacgaggtttacaccgtgttagccaggatggtctcgatctcctgacctcgtgatccactcatctcggcctcccaaagtgctgggattagaggcgtgagccaccgcgcctggccctatttatcttttataggacatggcttccagtctcaagttcagtttgtcacccataatggccaaagagcagtagtcaccttacctgtttcaggcaggaagggcagagggcaagaaacaaaatggtgctcctcctgattgagtcagcgttctttaaagatgttttccagatgttccacccagccgcgtttttttttttttgagagacagggtcttgctcttgtcacccaggctggagtacagtggcatgatcatggctcactgaggcctcaatctcccaggctcaagcgatccttccattttagcctcccaagtagctggaagtagctgggaccacaggcacatgccaccataccctgctaactttttcattttgtgtagagacaaggtgtcactgtgttctccaggctggtctgcagtttccaactcctgagtgcaagtgatcctcctgctttggcctcccaaagggctgggattacaggtgtgagccactgtgtctggccaagctacttctacttatatctcattggtcataacttgatcacacagccacatccagctacaatggagattgagaaatgtagtcttttggctgggtacacagcatctgaataaaatccaggcattgttactaaggaagaaggagtaagtgtcaatctctgctccataactctctaggttaatacacacagatggaggagattgctagttgcccctcaagatccagccttgccttctgggctaagaaagcccctgagatttacctggccatagtggcactgggaacaaacaatgtatttctaaatcttctgattttaaaatctttcagaatcacgatttctccgacatcagtatttttatgtctttagaattcaacaaaatgaaattcctaagtctaatatatgtgaatattaagttttagcagatactgctacataactttccagaagggtgtggcaattcacatctccaccagtgatcagcatgttcattttccatacagctctggatattttgtctattttaaaatatcttcttctaatctataatttaaaaatgtaacttagtaggaatttaattgttcatgtaaccaaatcttcccattaatggctatgggtttcttcttttacttcagaaagtcctccccaccttcagagtatataaacatttttttctaaattcccttctaatttcttataatttatagttttatttttgttatttgattcatttattctctcaacagatatttattgagcacttattatacgtcaggctctcttcaaactctggtgagagtattttctaactgggagagacaaccctagttgataagaaacaaacaaaccaataagtaaataagacatttcccccagataattaatacttggtgacgggggaagacagtgagacaggctactttacactggcaggtcaggaaaggcttctctgaggaggcaagtgattcaggattaattgatgactggtggagaagtccggggagtggacacaggtgggaacagcctggtgggtgtgaacagcaacaagaaggttaatgtggcttcatggaacagggtgaagatgagacaagctgaacactgaggtgggcaccagaacatggagggctttgtaggtcccaataaggagtatggattttattgtatactggagatttgtcatccatctagaatctgtttttatatataagaaaaggtgtatatgtttgcgcaagtgtgtgtgtgtgtgtttgggggggcggggtgggggcagacagggcgtaacttttctttaaattagagtcaaaatttaattaaactattcattctttacaggcagtgaggggattaggatcttatcccacagaatctcacctcatttcaaatgttgtacagatattatctgagatatattttcaggccgggtgcggtggctcacgcctgtaatctcagcactttgggaagccgaggcgggtggatcatttgaggtcaggagttcaagaccatcctggccaacatggtgaaaccccatctctactaaaaatacaaaaattagccgggtgtggtggtacacgtctataatcccagctacttgagaggctgaggcaggagaatcgcttgaatccaggaggtggagcttgcagtgagccgagaaaacgccactgcactccagcctgggcgacagggcaagactctgtctcaaaaaaaaaaacgaaaaaagaaatatattttcaatgaaatcaagcatataatgactatttttatcccagcatcttggcttcttcaggctgctataacaaagcatccctagtggagcatccctaatctgaaaatccaaaatccaaaacgttccaaaatctgaaaccttctgaacactgacatgacaccacaaatggaaaattctacatgtaaatacacgtaaatacaaactttgtttcatgcacaaattaaaaatattgtataaaattaccttcaggctatgcatataaggcatatatgaaatataaatgaattttgtgtttacccatgggtctcatccccaagatgtttcattttgtatatgtgcatactcccaaatctgaaaaaatccaaaatcttaaatatctgtagtcctaagcattttagataagggatattcaatcccttatccataaacaatttatttataaacaacacaaatttaggctttgtaaaaaatagaaatttggccgggtgtggtggctcacgcttgtaatcccagcactttgggaggccgaggcaggcacatcacttgagctcaggagtttgagaccagcctggtcaacatggtgaaaccttgtctctaccaaaaatacaaaaattagcagggcttcgtggcatgcgcctgttgtcccagctactcgggaggctgaggcaggagaattgcttgaacccggaaggcagaggttgcagtgagccaagattgagccactgcactccagcctgggggacaagtgagactccacctcaaaaaacaaacaatcaaacacaatataaatttatttctcatagttctgcaagctgagaagtccaagatcaagatgtgagcagatccacctttggtgaagggctgctttccatttgatagatggctgtcttcttgtgtcctcacatggtggaaagggtgaggcagttttttgaggtctcttttaaaagagaactaatcccattcatgtgggggtctgccctcatgacctaatcactttccaaaggccccacttcctaataccatcaccctgggggttaaattttcaacacacaaattggttggagagtgagcgaacatagacattcagtctatagcccccagggatgtagccactgaataaaataatctagaacttcatctagaggcagtttataagtcacataagaaaaccagttttacttatagtcacataaaacttttgataaaaaacaaccctagttgataagccatttgtttactggacttggctctgaagaaatgacttttggctaatcctcaaaatgaaatctactcacagagggcaagatctgccaccagtgaagatgtttaaaacaatgtgctgtaggctttgaaggcaagtctaaagaagagcttctaaaaatattttgcacaatggtagcattaaaagagtaggcacatgggccccaagataacatctgtgaagaggaggaccagtgtgtgtttccttttgtatgtttaagtactaagtcagtgattactttataattaaaccatattcctcttgatctgtccataataaggtcactctgtaatttataataggcttcttaccaaattcaagctttacaacaaccctataggttaaatattcctgtgaattttatagatgaagaaacagagtaagtgaaagagttcatactcaattcaagtctcttgagtctaaaatcagtgctctctctacataagaagttagttgctaagatcacacaacttgagaagagagaagacagttttcacagtccctcccctctgaccactaggctgcttggggtacttttacaacttacctgctctgaattaaggctctctgtgaatctgattcatctgccaatttgcaaacagtcagccctgtagtacgtacctaagttgatttttaaaatactatttctcatcttaaaataatggaaattgagtgacataaatttcctggacactttttaagatccaaagacaatttgctaatttgtcgttacaattaaagagccccccaaaaggcgtaagaactggattttgacttggacttctgttccttagtttctttaacatattgggggccgggagtggtggctcacacctgtaatcccagcactttgggaggccgaggcgggcagatcacgaggtcaggagattgagaccatcctggctaacacagtgaaaccccgtctctacaaaaaatacaaaaaaaaaaaaaaaaaattagccgggtatggtggcgggcgcctgtagtcccagctactcaggaggctgaggtaggagaatggcatgaacccaggaggcagagcttgcagtgagccgagatcgcactacactgcactccagcctgggcgacagagcaagattccatctcaaaaaaaaaaagaaaaagatattgggaaaactcacttaaactctatgggcttctgtaccactaaggcttctcaaatttgatgcaagtaatgggaacttgctgtggctaacttgagccacaggagaaggatactgcaagactcacaaatgcttgaaagtttcggaacaggtttggaaatgggtaagaaccaaggaccgggttgacctgaactgaaaggaaattgaggtgctattagggacaaatatgaaatgaaggatgaactgtctctgacatcctttgcttctgtgtttggagatgagtaagcagggagtgggtgcatatgcaaacagggtggtcagaaatgctttggccggatgtgtgactgaaggctatgtgcagctgaggaaggctgggccaccacagtagcagagaggctgaccaatttggcatgcagcaagcaggaagtagaagggatcttaagcaagcaaagtgtttgggtagacaagattatgaggaatgagcaccaatgacatttccaacaagcactgaaagcttccaaatgcttctaacagttactgcctgtacaaacacaggacagtcttgactatgtgagactgtgacagtttcctcatgcctatgaaatgagagacagtacttagcactgacatgagcttcatatttgaaggcagcaaactactgaaccacatgtagcttccgaaatcaaaagatgcaaactggcagaccacaggtcagatatgacatgcagaaaaaaattagttactatcttagcctagtttgtgctgcttacagaatatcagagactgggtactttatagagaacacaaattatttttcatagttttagaggctgggaagtccaagatcaaagggccatcatctcgtgaaggcgtccctgctgtgtcaaaacatggtggaaggcatcacatgggcaaaagagagagagggaagcgggggcaaactcctttttatcaggcacccagtcctgtgattcattcatgaagacagtgtcctcctggcctaatcacctcttaaagctcccacctctcagcactgttgcactggaaattatatttctcacacatgaactttggggaacacattcaaaccattacagttaccaaagataaaaatgcagatttcagatttctcttggggaagaaaaaaggctctggcaataccagggctgtatttccacatggcaacagttgtctgttgccttctgttgggttgtgggctctcacattgccataccctcctcatggcccccttcactcataacagtacctgcctagacctcgaagcactagtttccaaccctgcttgagttaactacttccatgacaactgtgcaaggccagagtgtgggcagctaccttgagggccaccggcatgggctgcccaagtgaccgagggcactaacctctgctctcgaaacttctttggtaggatctcttcactcctgacttactacttgtaactgctggaaacaaccatttattctacccctactaaaccacatctgtcttttctgtcagagccaatcttcaagcatatgcttcctcaaaagactttaattaccaggtagtagaagcggcagcaaagagtccccatctagcatcttctaaaatgtagtggagaaaccaacgacaacgaatctgagacaaccagttgtttgacttctctgaaaacaacctctaaaaaaagccttctctcgtgaatagctgcagacatgctgggcactaattgatgatgatgccctttagtgagtctcctctgcacatacctgattccatttggatgctggccctcacatacttctatctgcgaactccggaacacagaatatcatacaatgtatgattcaatctggactctgctggagccattctctacaaagcagacacaactttttcttgcctaaatcctttcaagttgctttatttttatttttaaactaattaccataaatctaatttatcaagctgcttttaagataaactttaaaatgcttagagcagtctacaaattcttgcactgtttcactcttccttatctctcagtcttcatctcccattgcatcttctctgactctttcatatggatcttctttcaatttgtggaagaagccaagcttgttcctgcctcaggtccttgacacttgctgttcactctcctgggagactcttccccccatcttagcttttaaataccagctggtcagactccttacctgccttccaccttcctctcattctcccactcctcgccttcatttctcagagtcctccgctctcttctttctattgctcttaacacaatttgtctgttttccgctaatctgtaaactctacaagagcacttaactattttgcatcccaccgaatattcggagtcagcacagaccccgtcataatagagtaggtaagcaatgcttacctgtcaaatgaatgaatgaaacacccgattcatcccccaagccagcttaatacattagatgatcttatggactgaataagacatccctccttttaaagaatatttttgttttagcttcacatcagcaaaccccgaacggttcatcctaagataagcctggtagagaggaaagatactaaccttctagggtcctaaagtggaactaggaacttattagatatgcacattctcaggcattatttccgatagcccagtcagagaattctgggggtatggcccagcaatctgttttaacaaacctttcaggtaattctgatacacactaaagtttgaaaggtttctttaaggctttccagttttcttttcttttttggagggatgggggggggtctccccatgttgcccaggctggtctcgaactcctagcctcaagctatcctatcctcccacctcggccttccaaagcattgaaattacaggcatgacccactgcggctcgcctccgtttctaacttaaaaaaattttctttggaggggagccttaatcctttctattatcctgctagtagaatcttactactcctgagggtaatctttgtcataatccaaaagccttgaataaaggcctatttgtatagttatgcagaatatattcctgggaggtttgccttcctaggagcacaggtcggccctgggaggtgggggttggggggcagggctgcattctaaagtcctgtaacaacgcacaagtacaactgaatagaactcggaacaaaggcatcagggccacggtgcaagtctttgttcatccgttccccgactgctcaccctgtctgataccgctcttttccacccagaaaagcagccactcaagttttaagaatggatgtatgccgcggacgttttcgattaggccgttttctctcaggcactggaggatattcgtggctgcaggaggcgcttccaccctttcctcaacctagcaaagaagtaactgaaactaacccaagggttacaaccgaaaagccccttccagcttcagaagcagaactggaagctcggatagacttctccgcctctacactcctggaaaacccgcagtggatttcaccaacttcaggatcggagcccaggcaggcgaacgtaccttattgcgcatgctcgctagcccctcccgctcggagcggaagggggagcgctgggggcctgggcctggcctggccggggcgtcggcaccggcggccatcttggcttcccggggaaaggcggcgtgaggggaagaagttgtagggtgggggcaggagtgaggaggagggaagagagagggggaggaggccgcggcggggcagggcggggactgcctgcctgcctgggttgcggaagtgatagccgccgaccgagcctgctgctttcttgctactgcttcggcttcccggctaccccccggacggtgaaggcggcccagctgtggatggtcagatagcccttgtctcccgccgccaatctctggcccctagcagcacggagcagacggcggcagcagcagcagcaggcgaggaggaagatggcgggacggctgccggcctgtgtggtggactgtggcacggggtaagggggcttacgggcgggggtggggaaactgaggcggaggaaggaagatggcgggggagggaggaggccgggaaatgaatggtgcggcgaggtgccgccgccggctgtcagtcctagacccgccggccagcgaggggtggggcccgcagccagggcctcgcgggtcccctcgtttctccctcctgggactggggcgggggcgcgggcccgagattcaacccccaaccctcccagcggctttctccgcgcgacccctcccggcccttcccccactacggtgggcagcgccgcccaaagggcgctggggacggtcgtcttgggggtggtccccgggcccgacccatccggctttcctttccctccgcgcccgtttttgccagtcggtttggggacccaggggccgagctcggggactggcctggcaggggagctagaaaagagaagcgctcctggtaggtttgacaagatcgctgtgacaacattctgcccagggtgtgggtggggaaagggaagaatcggactctgaaaatgggaacctacagtggggctttcatttgaccacccaccttctcctttcgactcctggtcatttccatctccctctgcgttttaaccggtgaaccaagtcacattttaattcgagggagaaagatgtcatgtgttacttctgtagcctcaaaaaagtcccccagtgagcaagcgcgctgcaacttccttagttttgtcaaagccgcttcctgctttcagtcttttatacccttataaggtagtttttagtttccaacctgagcacatcttactagaacttttaagcaggttttaaagagactgaattaccggtgcttggtgtccatttatatgacttaaaaaaatgtacttatgtttcatggagtgggggaaaggaagcaccctggaaaataaactaatttaagttgtattcgttcattctgtgatggtatcttgaaggaagcaggaaggtatagaggtatataggagggtgtttaagttgcaaatagttactcgtagatatgtagggtagtttgcgaaaatgtagagtggctttaaagtgtggtcgttcattttgtattaatagacgttttagagagttgtaccacactcataactgcatagagaatagactacccttatttttatgtagaatcactgcttcaggatgacatataggaaagtggtttttttttctgtgctgatgacatctctccaattcccagaacactcccagttttttttttttgagggggaagtc

SEQ ID NO: 19 - DNA, 26803 bp, Homo sapiens
gccgcacctaccgctggcctcagacatcagcaccccaaagggtatgttggagtcccatggtggaggtgccggccgctcctccacgcacttgatgtataccgaggatcccatgcttgacgtcgcagggggcattagccaggagcacgttgctgggatgccagtccaggctgaggatggtggagccaatgggcttcttgatgtacttgcacacccaccagttattctcccgctggaaataacagatggcgatgacacacagctgccgcccacagcaaacttgtcctgtgggcccagcacacacagcaggcagtgggtgcgggcttaccctcctggcccgtcagcgtccacacagaggccttgtggcctgtgccataggtcacgatgaggttactcttggaggcccagttgatgccttttacctgcccgttgtgctccttgagctcgggcaccttggcccacttggccccactcttacagcttcgtggttgttgaggcagatggtggccatctgggtgcggcccttgctccaggtttggcagcaatgggttcctgcagtcagctgtgggaggctgtagttgctctccttttcagagtaccccagctgcagactctgggcaggacgcacccaaccagtgctctggttttttgaagtaaaaaatgcataatgcaattttaccatcttaaccattttttaattatgaaatccggtagtgttaagtataattgtgttgttgtgaaacagatctccacaactttttcattttgcaaaactaaataactcctctttccccctactcccaagctccaggcagctaccatttctgtttctatgaatttgactacttatattacctcatataaaggggttcataagtatttgtcttttcttgcttggttacatcacttagcatgatttcttaagtttcattcatgttgtagcacatgtcaagatttccttttttttttttaaaaaaaaggatgaagactattcgtttgtatgtatatgccacattttgtttatccatccatttttcttcaaatgtttgagttgtgtgatgtttaattatgtgtcaccttgacggggcaaagggttgcccagacagctggtaaaacattatttctgggtatgttagtgaggctgtttccagaagagattagcatttgaattggcaggctgaataatgaagatctgccctcatcaatgtggatgggccagaacaaaccaaaaaggtggagaaaggaccagttatctccccaccacccctgtgccctttagctgggacatccatcttctgccatcagacatcagagcttctggttctcaggccttcagactccagaagttataccagtggcttccctggcttttggactcagactggggtttcactgtatgtttccctgattctcaggcctttggacttgaattgaattacagcatgaactttcctagttctctagcttgcatatggcatattgtgggacttcttgacctccataatcatgtgagctaattcccataataaatctcctcttatgtatctataattcatatagatatgatatctatatatcaatcccatagataaatagatgtctcatatatatatcaatgtctctatatgtagatgtctcatatatggtatctatgtatctgtatcatctctatatatctaatcatctaatatagatgtctcatgatatctatatagatatatctatatcatagatgcagagatatcatatatatgtctgtttctttggagaattctgactgatacaggttgcttccgccttttggctatcatgagtaatgccgctgtaaccatgggtatgcaaatacttctttgagaccctgctctgagttcttttgggtaaatacccagaagtggattgctggatgatttggtggttctacttttaattttttgaggaaatgccatactgttttccataatggttgcaccattttataatctcaccaagagtgcacagggtttcaatttctctacatccataccaacacttattagtgtgtgtgtgtgtgtgtgtgtgtgtttaatggctgtcctaatgggtgtgaggtgacatttcactgtggttctgatttgcacatctctgataattgctggtgttgagcatccttccatatgcttgttggtcatttatatatcatctttggaaaaaatgtctattcaagtcttttgtctattttttttccttccaacttttattttaggtctgggggtacatgtgcaggtttgttacatggataaattgtgtgtcatgggggtttggtgtacagattatttggtcgcctaggtaaatgagcatagtacctgataggtagttttttgaccctcccccttctcccaccctccaccctgaagtaggccccagtgtttattgttcccttcttagcatctgtgtgtagtcaatgtttagctcccacttataagtgagaaaatgtggtatttggttttctgttcttacattaacttgcttagaatgatggcctccagcagcatccatgttgctgcaaaggacatgatttcgttcttcttatagctgtggtgtatatgtaccacattttctttacccagtccactgctgatgggcatctaggttgattccatgtctttgatattgtgaatagtgctatgatgaacatatgtgtgcatgtgtctttgtggcagaacaatttacatttctttgggtatatatccagtaatggggttgctaggtggaatgattaattcacttttaagttctttaagaaatctctaaacctctttccccagtggctgaactaacttacattcccaccagcagtgtccaagtgtttccttttctgcacaaccttactaacatctgttattttttgactttttaatgatagccattctgactcatatgagatcgtatctctctgtggttttgacttgcatttctctgatgattagtgatgtagagcattttttcaaatgcttgttggccgcatgtgtcttcttttgagaagtgtctgctcctgtcatttgcccactttttaatgggcttgtttgttttttgcttgttaatttaagtttcatgtagattctggatattagacctttgtcaaatgcatagtttgtgaatattttctcccattccataggttgtttactctgttgatagtttcttttgctatgcagaagctctttagtttagttaggtactacttgtcaatttttgtttttgttgctttgtccattttaaaaaatagagtaatttgattattttgttgttgaattgtaggaattctttatatattatggatgctaacatcttatcaaatatgatttgcaaaacattttccctcattctgtaggttgccttttcactattgtgtccttcaatgaacaaaagtttttatgtttgatgcagtcccatttgtccattttttttggttgcctgtgattttggtgtcatatccaagaatgtggaatgtgtcatatccacattcaatgtcctgacgatttttttctatgttttcttccagaagttttattgctttgggtctttggtttaagtctttagtccattttgagttaatttttgtatgtggtgtaagaaacaggtccaactgcattgttttgcatgtaaatatccagttttcccagcatcatttgttgaccagactgtccttttcccatttagtgctgttggagctcttcttggaggtcagttggccatgtgtacacaagtttatttctgggctctttattctgttctattgatttgtatatctgtctttattccagtaccacactgttttattcttctttttcaaaattgtttgactcttagggccctttgagattccatatcaattttaggatgaattcttctatttctgcaacaaatgctattggaattttgataaggattgaattgaatctgtagactgttttgagtgatattaacatcttaataatattaagtctaatccatgaatgtgagatgtttctatttatttatctcttctttgatttctttcagtaatgttttatagttttcattatataagtttttacttccttagtcaatttctaagaattgttttctttttgatgccattgcaacgggaatcattttcttaattttttcagatgctttcactatttgtgtatagaaatgtaactgattttttgtatgtgtgttgattttgtatctggtaactttactgaatttttaaatttgttctaacctgttttttttttttggtggaatctttaggattttctgcatataagatcatgccatctacaaacagaaatttttacttctttcttcccaatttggatgccttttattgctttttcttgtctaattgctttggactggagttccaatactctgttgaatagaagtgtccagaacagacatttttgccttgttcttaatcttagaggaaaagcttccagtttttcactgagtatgccgttagctgtggacttttcctaaacaacctttattatgtgcaggtaatttccttctctttccacttttgagtgttttttttcttttcttttctttttttgtgtgtgaaaggatattgaattttgccaaatgcttttcctgcatcagtggagatggtcatgtgggttttgtcctttattctgtaaatgtggtgtactacattgattttcatatgttgaaccatccttgcatcccagggataaatcccacttgatcatggtgaatgatcttttgagtgtgctgttgaatttattttgctagtatttttttgactacgttcatcagacatattgggtaattatttattttttcttgtagtatttttgcctagctttgatatcacactaatgctgcccctcaaagaatgaccttggaagtattcctttctcttcagtttttgggggattgatgtaaattcttttttttttttttttggagacagggtctcactgtcacccaggctggagtgcagcggcacaatcatagctcactgcagcctctaactcctgggctcaagcaattctgcttcagcctcctgagtagctgggactataagcatgtgccaccatgcacagctaatttatatatatataatataatagataaatatatatatatatatatatatatatatatattttttttttttttttttttttttttttttttttttgcagagacaaggtaggtcttgctatgttgcccaggctggtctcagactcctaggctcaagtgaacctctcacctcagtctcccaaagttctgggattacaggcatgagccaccacgtctggccagtgttaattcttcaatatttggtagaattcttcagtgaagtcttctagtcctgggcttttctttgttgggaggtttttaattaccaactcaatttccttactagttattggtctatttatatcttctatttcttcatgattcagtcttggcaggtttggtgtttctagaaatttatccatttcttataggtcatccagtttgttggtatagttcatagtcttctcttataatcctttcttatctgtagctcagtacctcctatctggagatgcagaattaggaattgaaactataataggccccccttttataatggggtgtccttatttttaccttctcaccttgcaatacccttgtcttgctagtaaagaaagaagggaaatttgattcaggaggtaatcatacttttcaatttgtacaagatctaatagccatgaactcctatgtcattcctcaccatcccataattcttagcccagccatcatccttacctcaatccctgctggtgcagcctggtttattctgttaatgtgctgtactgcattgaggtaaggacttctgctcagctttcttcttgataccattgtaccttgattcacacttcctcttgtgaaataaagtttagcatgaagctgctttcttacatattttaagttcggcttaaaggtttttctgtacatcgtgaactgtaacaagtggaatataaccagaccgtagcttacacttgtgccatttaccaagttttggccaatcaaatgtagccaactgtttgaactgtattcaaataagggaaatgctcagctgtaaccaagccaactgtttctgtacctcacttctgttttctgtatgtcactttcctttttctgtccataaatcatcttccatggcgtaggtgtgctggagtctcagagtctattctggctcaggaggctgcctgattttgaatcattcatggctcaattaaacttctttaattttttttttttttgagattgagtttcacccttgttgcccaagttggagtgcaatggtgcagtctctgctcactgcagcctctgcctcctgggttcaagcgattctcctgcctcagcctcctgagtagctgagattacaggcacatgccaccatgcccagctaatttttctatttttagtagagacagggtttcgccatgttggccaggctggtctcgaactcctgacctcagcctcccaaagtgctgagattacagatgtgagccactgcacctggcttcactccttcaaatttaattcagctaaagtttttatttttttctctttcttttttttttttttttttgagacagagtcactgtcacccaggctgaagtgcagtggcacaatctcggctcactgcaacctccgcctcccagactcaagcgatttctggctaatttttgtgtttttagtagagatgggttttcaccatattggccaggctgatcttgaactcctgacctcaggtgatctgcctgccttggcctcccaaagtgctaggattacaggcatgagccactgtgcccagcctcaaatttaagaagaaacagttaacatggacttgcatacctccaggatattgtgaatacctctcaatatttttctaagttctcaaagtcaaattagactctatgacaatcactcaaggttccctttgtttccaatatgttgatgacctgctactttgcaaccaaagcaaacagggtgctcttctggactcccttactcaccttaaggcactgactgactaaggttataaatcttccaggtccaaatgccaacaggtacaaaaaattcttacctacttaggccataaaatattttagggtactcaaaaactcgtcccaaaatgccttgaatcaattttattcattatctctcaaagacaaacaattacgtgaatttttaggagcaactggatattgccaatggattcccaattttgctgcccatgtctaacctttatatgctgtcctcttagatacaaccacagagcactttacctggtactctgaggcaccagcctccttggaagcattgtccacaccccagcccttcgactacccaactttgacaatcttttttacctatattactgtgaaaatgatgggattgttgtgggtatcttaggacaatctttttgtcccataacatatttctcatgtcaacctagatatgtcccacagtacctttctcatgttaagtagcatcaggcattcctccatgcttatatgcaatagacttagctgccatcctaattgacaaagcaagtattcttatactgccccaccattcacctctctgttctccatgctgttcctctacattggtatccctttcaaagtggatcttgcctcaactaacccttaactgttttttttttgtttttgttttttgttttttgacaattctggcactaccccaacacctgcttgttccaatctttcaaagcctggccaccttaaatagttaatctggttactggttaggttaacatctacataatgcagaagagtttttgttcctaccaatgtaaatatacctggtgaacccattctggacaatggatatataaaagcatatggtatccataagcaggaagacaaagtcactctgtctcctcctctggtagattaatttggcactgggaagcctccatggaagctcaaggtcagtgctttacccaagtaagactattggaaggaaatctctctacattgaaaataaatacagtactggaccttttctgggtaacatttcaaaaatgtattgcaatcaaattctgtgatttggcttcacagatggcactaaacaaccctccactgtcattgttacttggattataactaagtatttcaatgtgagtgaatgtcagattacaggataatattcctggtttgtaggaaaaagtagtgggatatggaatagctcaagtgttcccctagttggcttgaccagcacccatgactatagttggatggatggaccttaacttggtcaataaataaaatacatttctatagtaaccaaggctaaattaaagggtttctctgccaggtgtttcacaacctgttttaccctcatagcctaacagaagcacattggaagtgaagatgtgcagatgccaacatgattgatgataagggttgtgaaagacacagaattccaacttggttgttcacaggttccaccactatgaccttgtctgtaaacaacactggtctctctctctttttttttttttttagaaggaatctcactctgttacccaggctggagggcagtggcacaatctcagctcactgcaccctccaccttccggttcaagcgattctcctgcctcagtctcccgagtagctgggagtacaggtgcccaccaccatgcccggcttatttttgtagttttagtagagacaggatttctccatgttggccaggctggtcttcacctcaagtgatccgccagcctcggcctcccaaagtgctgggattacaagcgtgagccactgtgcctggcctggtctcatttttatgtagcaataagatatataaaaggttcccacctaagtggtcagagaaatgtgaagttggatatctggtgccttcccttaccagatatcccactttgaatgctagccacattacaactggggttcttttatatataaattaatgccatgtagatgcacctgatgagacatcatagacaacgcacttatgtattgcaaccctaagttctcagtaatgagaatgcttttccaaagcctggcaatgtacgatgtagaaagaacaatcctaagcattccaaagtaatgaacaagcatctggtgccactatacagactgggaagcctgccatttacaagttagcagtgtagcctctgttgcactccaaaattgtgtcctagatatgctgactgcccaacagagaggagcttgtacaatcactggcaacaatgctacttctatataaattagaaaggaaaaattgtgtctaatctatatcatttaaaaagaaaggttggccgggcacggtggctcacgcctgtaatcacagcacttcgggaggccgaagcgggcggatcatgaggtcaggggatcgagaccatcctagctaacatggtgaaaccctgtctctactaaaaatacaaaaaattagccaggcatggtggcgggcacctgtagtcccagctacttgggaggctgaggcaggagaatggcgtgaacatgggaggcggagcttgcagtgagcagagatcacaccactgcaccccagcctgggcgacagaacgagactccgtctcaaaaaaaaaaaaaaaaaaaaaaaaaaaaaaaaagaaaggtcaacattctacgttaggtaaataaggcatagtccaattaactgaactgaactgacctattcccacgactgggagactggttcaacagaatatggaccagtgtgttcagatttttctctgttgtaatctatgttcttctttcattttgcagatctcttacctcccagcacctaatatgagtcttttctacataggaaataatccaaatatttgtgaaacttcatgtgaagtttcaaatgggggaagtgaaggaacgaacaacccacctcctaaccccaatttatacccacctgtgttagttcatttgtattgctatgaagagatacctggaggctgggaaatttataaagaaaagaggcttaattggctcacagttctgcagggtgtataggcatggcatcagtatgtgctcagctcctggtgagggcttcagggagcttacaatcatagctgaaggtgaagggggagcatgcatcttacatggtgatagagggagcaagagagagggtcggggggtgccaggctctttaaacaaccagctctcatgtgaaataccagagccagaactcactcatcaccatggggatggcactaagccattcatgagggatctgcctcatcacccaaacacttcccagtaggccccacctccaacttggggattgtatttcaacatgacattttgaggggacagatatccaatattcaaaccatatcaccaccagaaaggcataaagattactttaaactgaaaatattggaacaaacaatcgctgcggaaagcagccttatctgaccgaaagcagacctgtccaagagttctgctatcatcaactccttctgagggactttccagacagcgaggtgacagatgtttacaaacgtgacgttaaaaaataaagttgtgtaaatgagtcttatcagaaccttttatactttctcactgaagcctcagttggtatataaacccttaccactggctgtttgggaagtgactccttacagagtgctccctcaggcatggagaataaacttttctcctgttaatgtattttcaactaattcgcaggccctagaccactcagatctaagttgacagatgaaatgttttcctcccaacatgaccaagcttatagtgcttttatggtatatctgtagagattgcggtcaggcataacattgtttgttagggttgcagtacctttcaggaaatgctcaaagtttaattgatttaggggactttcactggatgagatgcctctctgagtcatcataggttgcaaagtattagttttttgccactcactgtgtgttgtgatatgacatactcataatggggtaggacaagatgtcagttttgcttccaaactttccttacttgtttcctttttggttcaccactaatgttgaagaaatgcaagatggaaaatctcaatagttgacactgattgattgattgagatggagtctcactctgtcacctgggctggagtgcagtggcgtgatatcggctcactgcaacctccacctcccaggttcaagcagttctcctgcctcagcctcccgaacagctgggattacaggtgcccgccactactctcagctaattttttgtatttttagtagagatggggtttcaccatgttggccagactagtctcgaattcctaaccttgtgattcgcccgcctcggcctcccaaggtgctgggattacaggcatgagtagttgacatttattaagtgtttatatgtgataagcactgttagattatcccatgtaatacatcacttgattgatttaagagattgtcatttgaaagattaaagaatatttcccagaaaggatgcttggtcaagcctcatcatcctgggatggatgggaccttggttttgggcaagtttattacaatttaagactattctaggtcatggaagtgtgtgttaggacatataagtagttttcttgtccagaatactttgtaataatataccctaagtttgatcagctttttggcattcacttaattaaaatgttcacaagtaggtacatttttagaattgttaagtaatatactatttgtagtagcaaaacactacaaacaaatacctaatataataagagggagtggttgaataaactagggcatgtcaactaaaaaacatatttgaaatgcagggaaaatgcttactctaggcaatagttacaacttttgtccattataggtacataaaggaaaagagtacacaaagaattctattaatgatgaaattaggaacaatgttcccatccccaatttatacccaaaagaaaatatgttctggctgggcgcggtggctcatgcctgtaatcctagcagtttgggaggctgagacaggtggatcgcctgagctcaggagttcaaaaccagtctgggcaacatggcaaaaccccgtctccaccaaaaatacaaaaaattagccaggcgtgatggcacatgcctgtaggtccagctacttgggaggccgaggtgggaggatcgcttgagctcgggatgtggaggctgcagtgagcaaagctcacaccactgcactctagcatgggtgacagagtgagaccccgtctcaaataaataaataaataaatgaaaacttatattctataacatgtattcttatgtctttggctaaaacaaaagagaagaaaaataagtagagagctaagtgaagtgaagtgtcttgaaacagataagccataaagtgagatatatgagtaaatgagtagttgctggcctaggaattgtttctgatgttttcacctattgaaagaatttttttctttttgtaaatcttttttttggtttgttaaactgaaaaataaaagcaatgaagagataatattgctgtagtaatgtcccttagtgcatccttggagttagttgtcttgaatttggcctgctctgattgtcatttgctgtttgctgcattgaaaaaatttcagatttacaaaaatatgtgtgccagggtggaggaaatttttaacttgatgaattctcacctttaggacactgtctgctcttatatggcacttagcaagatgctgcaacaattgtccctgctcatactgttggaggaagagggtatttgcagggagattgctggagtcaagatgatccaaatttaaattgcagtggtgagcagtggccactagagggctgtgaagtacttaattctaaaatttccacattttaatctggagcagaggaaactctggaaggaccactgggactaagggagctcaatcccaaacatctttatctgagccctaaatgtcttctacgttattctttgacaatactttgttacatctcagaatttgtagttttgaggtggaggtttaagttagaaatagtttaatatattctattccagaatataattcgcttttttccaaatgaaactggcactaaaagctttttacttgaaagcaaatacacttcatatgctttatgtatttttgtccctatatcattgaaatagtagattcaaggctgtttgtaaaaataagtgactatactgcatataggaatagccccaccttaaagactttgattttaaggacattaagtgggagggtcttttttgcctttttttttttgactatcaaaatactttcacatttcttcaattcaaagaacaactgttctaaatttagaagacagacaagtgaaagagaatatgctgccatttccgatggttcttttttactcttgatccatcactctcctgtctttggctgactctttctccaaaaagtaccccttatttttcctatgcctttaacttctgttttacttactctattgtagaactttgagaagttgtacaccacattcactgctacctcacattaactctgcttactcattgcagtctgccttctgctcctcaatgattgctcctgtgaaggtcatctttggtttagcacttgtttgaaatctaatagcctaaatgcacatcgattactgtttagaattcaaacgacatttatttatttactttgagatggagtttcattcttgtcgcccagctggagtacaatggcatgatcttggctcactgcaacctccacctcccaggttcaagcgattctcctgcctcagcctcctgagtagctgggattacaggcaccctcaaccacgcctggctaagttttgtattttttttagtagagatggggtttcgccatcttggccaggctggtctcgaactcctgacctcaggtgatctgcctgcctcagccccacaaagtgctgggattacaagcgtgagccaccacgcccggcccaaatgacatttatttttaaaagcaactaaaccaggaaagaccttcactcattcaatcaaaaaacatgcattgaacacgtattcttggctagatccggtgctgcaaagatgaaagacgccactcctagcctcaaggagcttgcagtttagtggtggcactggatgtaaaataatcataagatgtgaggtgaagactgatgaggtctattttgttgacacaggtaaacattctcagagaatatttaattagcaacatgacaaaaattagttgatttatttgaaggatatttaagtgaatttagagatgagatttgtttttacttttttaatttcagagagttatgttggttgcaaaaatctttgttttctagtatctattttataagccatctgagaccaggatgttttctttttaacatgtaaacttgatgcagtctctttgtaaagtaatgaatccccccgtgaacctcaaggagaagaaagtttagcttgaacacttaatttcaagtaccttgagaagggaacaggctgtattgctcagagaagaaggctctattagctaaggtagaaggacaatgtaaaactcttgtgaagacacctaaatgtcattccactcaaagcccattattaataatttgaaactgtctgctctgtgaaggcaacgacctatctttactcatttttgactctgctaacatttctttttatagttgaactagaggcaaggcaaggaacttgacatgcttgttttccctttagaataaagtggccagaagcagtttcttctgtgtgatccaacactttcttatccccagagcaactctgcatagtctagatgtaccagagcccagcagcctgtgaggtgatgtgatgtgatgtgatgtgaacagaaaggctccatgttggatgatgcctatgaatctaatcagattctctttcttggtcattttgatttccagagaaggcagtagaagcaggttctgtgtgtataaccagagactagagggaggaactgacagggaagctgggtcatgagagtggtgtgctcagcagagtagggagtaagagagagctggctccagagaggatgacaaaatgcccatgtctccagcacttctttagcattctgagttcccatcctatcatgaataggaagagttttctagctctccatgaagccgaaataggtttcagactttcctttctttcccacacacataataaatacccatcaggtaacctgggcatggccttttatttaggcactaacaattctaaaaggaattaataaatgcttcactgccatttcacagtgtaacagcatgccagtttaccataccattaacatttagcctcgtggtatttctgtgttttttcagtcagtaatgatggcatttttgccaagataatatagtgttaaactgtattggttgaaatcctaggctttttaaatgtaaactagcactttacaaagtattacaaaggaaacgaaccagggaaacttgagaaggaactttcttatccacattgttataggttataaaatagttcctatttaaattaaaatacctactgttgcacttttatgtgtgtttttatatataaataacatctgggttggcaaatatgtgattttcgtcaaataggctttgattgaagatgaaatatttttgtaaaactagtccttttttaaagttaaaattttatgttaccacatgaattgatcagcagaaatttatttacattatgtaaattgatttttaagagtatccacaaggttttagctattatttttgaacttgcttcctagcccacacaattaagtaataagagtaagaaaaaagaaagcacacatccaaatcatctatcaaaacccagcttctacccaatgacacatcattttatttcttgatcttgtaatgttgagcacatgccttggacatattcctatatgtgggctctattctctgcagcacgtcactccctcttttatccgcccctcttatgtgctcccactcctatcctcttcaattaaaaatgcctctttcttttttttttaagttaattaattaattaatttttttttattgatcattcttgggtgtttctcgcagagggggatttggcagggtcataggataatagtggagggaaggtcagcagataaacaagtgaacaaaggtctctggttttcctaggcagaggaccctgcgggcttccacagtatttgtgtccctgggtacttgagattagggagtggtgatgactcttaacgagtctgctgccttcaagcatctgtttaacaaagcacatcttgcatggcccttaatccatttaaccctgagtggacacagcacatgtttcagagagcacagggttgggggtaaggtcatagatcaacagcatcccaaggcacaggaatttttcttagtacagaacaaaatgaagtctcccatgtctacttctttctacacagacacagcaacaatctgatttctctatcctttccccacctttccccctttcctattccacaaaaaccgccatcgtcatcatggcccgttctcaatgagctgttgggtacacctcccagacggggtggtggccgggcagaggggctcctcacttcccagaaggggcggccgggcagaggtgccccccacctcccggatggggcggcggctgggtggaggcgggcccccacctccctcccagacggggcggctggccgggcgggggctgaccccccacctgcctctgggacggggcggctggccgggcgggggctgaccccccacctgcctccgggacagggtggctgctgggcagaggggctcctcacttctcagacggggcagctgccgggcggaggggctcctcacttctcagacggggtggccgggcagagacgctcctcacctcccagacggggtcgcggctgggcagaggcgctcctcacatcccagacggggcggcggggcagaggcgcttcccgcatctcagacgatgggcggccgggcagagacgctcctcacttcctagacgtgatggtggccgggaagaggcgctcctcacttcccagactgggcagccaggcagaggggctcctcacatcccagacgatgggcggccaggcagagacgctcctcacttcccagacggggtggcggccaggcagaggctgcaatctcggcactttgggaggccaaggcaggctgctgggaggtggaggttgtagctagccgagatcacgccactgcactccagcctgggcaacattgagcactgagtgaaccagactccgtctgcaatcccggcacctcgggaggccgaggctggcggatcactcgcggttaggagctggagaccagcccggccaacacagcgaaaccctgtctccaccaaaaaaatacgaaaaccagtcaggcgtggcggcgcgcacctgcaatcccaggcactcggcaggctgaggcaggagaatcaggcagggaggttgcagtgagccgcgatggcagcagtacagtccagctttggctcggcatcagagggataccgtggaaagagagggagagggagactgtggggagagggagagggagagaaaaatgcctctttcaatatgtaaggtaagattgatagatgattgccttccgtagttcctcccaaaattcataggttgaaatcttagccctcagagtggtggtattaggaagtatggagcctttgggagataattagctcaggagggtggagccctcccgaataaatttaatgcctttataagcaagaccccagagagccctttcacccttttctaccctatgaggacacagcgagaagacagctgtctgtgaaccaggaagcaggccctcactacataccgaatctacaagcaacttgatctcagacttcccagtctcctgaactgcgagatataaatgtttgctgtttaagtcacccagtctaaggtatttttgttatagcagcctgaatggactcaggcggtaggcaagaggaggacagtgcacctgagttatacattgggcaagtcatttaccttcattggagcctcggtttacttgtgttagatatgggaataatgatagttacactgcagggtggttgtgaagattagagaaagtgcatatactctgatcagcacagtgcatggtacttcagtacacagtgttaactgaagacacagtgttaactgaagacacagttgaaaactaaagatagctagtgaaacacatgttctctgcacatcatacagtttcttgggcagttttcaaagtgtgactctgcagttcataccaccattatcacttagtctctaacaaataatcatatttgacacatttggctgggacttaataattttatttgggcagcagctggtttctggaagtgttcatgggaagaaaatgtatattaataaagttagcaggtaatgttctttgttgaaatgttggatattgtgggacacaaaagagtcagggtaaatgtacatttacagaattgagcgtcagagtgtcatagttctctaatgatttacaaagaaagaattcctggaacaagtgaaatacttaataattaattcagcctgtatttctgcaggtaatcaactgcagtgataaaaaaataaaaatggaactgtcttttgctcattggaaagatatttgctgcattcaaagtcatcaaaaaggcgaagcaatgaaacttaagacttttgggttttaataattaaaaatccatcttaaagagaaccttgggctctggcacggtggctcattcttgtaatcctagcactttcggaggcccaggtgggcggatcacttgaggtcaggagtttgagaccagcctggttaacatggtgaaaccccatctctactaaaaatacaaaaattagctgggtgtggtggtgtgcgcctgtaatcccagctacttgggaggctgaggcacgagaatcacttgaacctgggagatggaggttgcagtgagccaagattgtgccactgcattccagcctgggtgacacagtgagactctgtcttgaaaaaaaaaaaaagagagagagaccgtttgtgaaggtgtgttacacagagaattcctgattcctaatctccagaatagaaaaattcaaaggctcagaatcatcccaaatcaattatccagtggcatctgcattttccgatttcattctcactagccgtgtgaacatgggcatgaccccaggagccaaggaattctctaatgcctaaggacagccatgaggtcaatgaataacatgtgtcaggtttccctggcacagaggagcttcccagtaaatgttattttccttagctatttcccatttaacatgtcaattattcttagtgagtttccattcaatatgagagtttatataatttgtcatattgaataggaacttgctaaggaaagctgtgtagcagaggaagcagccccaagtgacaggacataaactttaaattcacaagatgcttgtatgtgaattatgatggtatctgaattaacagtgatatttacagtttagtaatacatttttcttcccttgtcttgggctttataaaaaccctgtaagtcatgtatgtcaggaattttatcctcataattgagagaaaaatactccatattttattggaaataagatcagtagattctctgtatatcatacaatgtcttgcctacttaaattatcaccccccttcctatttcaacaaagactttctctaagtacccctggcctcttgccctgatccatactgttctccttggtaatggagtgagtttcctgcctggtgggtgcagccattggccacatttctctagtgtatggaactcaccggataaaaggcctcagatgtaggtctctttctgctgtcttcacccaggtgttgtggagtgtgtctgtccttgagcactagctttcccctgtgtgggctgcctcaaggcctgcattcatcaggtagggactgttagctggtagacctaagccaccactccagtactgactgtcagtaaggaaggtgacatgctgacctccatctgctacatcattgtgtatatgtcttcattagttctgcatattggtgagaaaatggatgctctgattcctcttgaaccccaagagaatgaaggtaaaaaaattgaggtcctaatgcaaattttcttagtacacccaaatctttggatagagtcctgcactctttgagatatatcacacaatctgtctcactttcttttcgcatatgttatatattttaaaacttttgtttttggggccaccacttactggctctgtgattttaggaaagcttttcagaccctcagaaccccagtctcttcatctctaaagtaataaaatatatgtaaagaacctatttcagcatgtgaattctgttttcctttttcctctagatgtatcatatccagttaaaaaaaaatctacttgaactttgcaggtatcttcagtgtttattacttctcatttttaacatttattggaaattagcatattgtcagaattgatataatacaatatgtaacctctttcattaagcttatcatttttaaaatacaaataactattctttacttaaatttttatttctagacacagggtcctgctctctcgaacccaggctggagtgcagtggcacaatcatagctcactgcagcctcaaactcttgggcttaagtgatcctcctgcctcacactctggagtagctgggattatagacctgagccatggtgtccagcatgacttaaattttgaataagttgcacttactaattacacttacactgctgcatctgaaagagtaatacaacaatagaagccttttatagtaattatttgtggcaggtagactcctaaaatgactcccaaatgacccacacccttgtacaatcaataccctgtcccttgagtgacagtgacttgctctaatcagttggctttcagttaatcaaaagagagattatcttgggctgaactaaactaatcccagcaagataacagggacttcagtcttgcaaacagatatcatataaagggaatcatatctgcacatttgattcttggaccctgggtaggaatttgttagagagcaaggatgtgaataaaggtgggaaataaaggtgtatctggtgtctctgctcaaaagctcacatgtagctacaaggcagagatttaggggagtggtatccacagtcaagaagaattaatacatagtgtttgagtctggcttcttccaattagcataatgcttttgaggttcatccatattgttgcattaccagtagtttttatttatttattttatcagtagtttctaaattgttgagtagtatattacattgtgtagatatatcctgtgtgtttatccatacacatttatggatatttgggagttgctagtttttagctattctatgagcattcacatacatgtctttgtgtggaaataggttttcatatctcttgggtaaatatacgggagtggaattgctagatcatatggtaaatactctgtatacttaaaatgaagagaaactgtcaaactattttccataatggctctaccatacttgatgttttagaaaagaggaaaaacactagcaattttgatgctgtatgtctacaacctaagagaatctaataatagcgtcctggtctgtcagtgtaggaattgcctaggtaatacatggaaggtgtggagggagcaggtacacagaaaatgtgcgtcagaaagttttgcttttcctatcccacgtcatttctgagtctgatcctccctactcctcacaaataaattggtagattcatctgtttttggacccttttctgctctagttactgaactatcagagacttcaggaagagcttaagctaagctattccagggaagttttggtgttactctgtacttacggactcctgcgtgtctgtctctgtcaccccagctgccaactcaacttagagtttattagcctggcattgaccagcacactgtgatattctctgaggcacactgcatgctgctagtgtgccctggttcataaagctgggccttcagcattgatcccactccaagttccttgctctgtcttcccacagctgtccccttgggggatgtggggggtctgacatcatttgcattattagtctattccaagaaatgcacctgtgcactaatcagttcactttttctgtcttagtcggcagatctagccatagcccaatccctcaatttctatactaagccttttatattagtaaaactgttatgttatctagaaattcatcagtgggaaaactacttcaagggaggtagttagaggctgcaaggtgctaaatatttttctttctttctttttaaatgtaacttggatctaaagtaaggacgaatttccttttattatttgttcagaatataccagctggtcctgtgggcagaagtttgttaaggggcctggatgtgaaataacagtgtatctcgtgtctctgctcaagagctcacatgtagctacaaggcagagatttaggggagtggcatatacggccaactgagaaataacaatattgtcagggactccaaggcactttggaagatataaagaatttcttaaattttcttgtagaattgttgcaaaaggcagacatgcttaaatgtttaaataagcttcttgaaaactcatggaacattcaatcacaactccaacagttctccaaaatttgatttattctggccatattatgcagcaaagaaacacttggctatttatctaaatctcttctgtcttgtaaatgatcctagaaaataatctagaaatacattttattaaagtaatgcatgaggtacatatcgattaccagccaatagttgaacttaaacataatgcatgggtgtgagggctggcattgatgattcacaatgaacacagttgaatatcacttccctgctgagactcgggtatcatcgcaaaaccacagtgagcatcagtggggatctgcatgctctggtcaagacagatctccatgctgagtgtctgtttgccatgatgaagagaacagtcaacaggagtgtttgccatgatgtagagaacagtccgggaggagtgaatggaggatgggggcatgaggaaagatgaggctttctctagttatgaccctttgtgtagaagttaggagtaggggataaatgtttctgcctaatatttaacttggaagagaagatgtccatgtgaaaaactgctaaatactgaaacaagagagcatgtgactaagcaataccatgtgtggcacagaaaacaagtgcaatagcagtttagcaaagtgagttcagtgtaggctgaactggttagagcaggtttccgggtgaaggtgaggattggtgagggtttggattggtagaaagagacggggaggacatctcacatcaagaagttatgccagtggatttcaggagaattgagtgtttgtgtctgaaaagcctgtaagaatagggcatgacagtgtggagaaatgcatgaaagtatgaaggatcgtgatatccagtttgaggagtgctaactagaggctctgaagatttgagaagaaacataatgaaaggtgttctcagcctgatcttggtatgcaggactggtaaaccccaaacaccttaccattctattacctctccctcaaggaatgggtcccttgataagaatttagtgtaaaaaagattgtcaattcagtgctgctgctgagtgctagtttctttaaacacacacagttttcttttgagaattttttttctattagatagacgaactgttatttaaatgaaaaaggcacatagtcccataaaacaattacacattcgggtgataacttcaaaaggagaaattaaaatgttcttatgttttgagcaagcatttccacttccagactttgctgcataaacatctgtggtcatctagggaatgcctgacctggttcagaggtgtcagagcaatgtaaagtcacggaagtgctgcagttctattctgggctctcatctttttgcagcggtccattctctaattttcaaccacatattaccagacaatctcttaagtcatacacaacaaactgattctgtttcaatgcttagaattagaataaaaaagcctaagcaaaaatagcacaaacatttgaaaaacactccttttttctaccactcccttcttagaacagaaataaaagccctgtactttaagaaaatggatggaagaattttctttgtacttcttattctccaagttacatttactacctgatagtgttaatacctttttgtagtacctttctttaaaatatacagggaaatgatctgttccaagaaactgtgtttttaaatttaattatagtgtgctatgatgatttaaaaaatggccttttgagtaaaggacacgaacaagttatttaaaaagtgagcagtaagtgtggtcagtaaacacatcaaaaagttcccttcactaatattcaaagaaatgcaaattagaataataatacccttgttgcttgtcaaattaatactttaacaattattatgtaaattttatggataggattgcaaatcaacacacctttcctggccactggtgtacataatagaaattctaaaaatgttcttaggcttgaccaagcatttccacttctagactttgctgcacaaagatctgtggtcatctaggagaaggcttgacctggttcagaggtatcagagcaatgcaaagtcatgaaaatgctgcaattctatcctggactgtcatcttttttgtagtggtccattctctaatttttcaatgacgtagtaccagacagtctcttaagtcaaatgtatttgtagggctctggatttgaaattcaatctggctttcagccttgatgtggccactcccaacttgtaaaggacctgtgaagacttagacacagaataaaacacagaagataagaaaaccaactttgaaagaaaatttattgtcaaaattgtactgggtcaattgagcaaaaacttcaaagagcgttttcatattaaccaaagcatccctcctcaattgaaacatataaagatattgttcacccctatcctgactcagagatccacaaatctgggcattcatcatcaccatattctgctggcaatagttttaagcagctaaattactgttctctactcttgagtttcctccatctcttcagatacagaaagttctagaatatattcaaataatcaaatctttaattcattccatatatctggctcaagacagtgtcccaataaccttattctagagaaagtcagatttagacttgtgctcatcatcatactcatgttcttgacatcattttaagctctgaggagacatctcacataactctcattgatacgtgtatacatctgtcactctgtgtttgtgctgtgatggatggacttggatgtagatatgcatagatgatgaagcagatagctatatatatggtattgatgtagattcagtacagctgtataattgcatctgtgtttcacatatcttgtgtactgtatcttgactgtatctgtgtcaatacctaattgagttataaggcataaatatgtggagctcttagcacaatacctggcacactgcaatcagtcgatgtatgtgtttgtgtgtgtgcgtgtgtgtgtgtgtgatacagacagaacctgctaatatgcataatagtcaggttgggttgttataacaaaatactatagactgtgtggcttaaacggcagacatttgtttctcacagttctggagtctgggaaatccaaggtcaagattagtttctggtgagagcagtcttcctcttttgcagctccccatggtttgcaaatcacagatttctcgctgtattctcacatagtgtaggaggaacagagggagggaagggaggaagtgcctaaggacactaatcccatgatgagagttctatccaccatgacctaattacctcctaatgccaccatctccaaatactatcacactgggaattaggtctttaacatgtgaatcatttggggtggagaagacaaacattcagctcataacaggtaaggtagaaaatctcaagaatttatattttgtatatgaaagatcattaatgagcagaattttaagtttaatgccaattttaatctatttttatcttttctacgattcttttttactttttaatttttaaactttcatatacaaagggataatatttggctaaatgttctcttctttttgagctctggatcattgttacgatcaccccataattgtatgtgtgcagagatagtgctttatacatttttaaaacaattttatatacagtattaaattttatttttcaataaacaatccatgagatagaaagaacatatattttgttttacagataagctccagggagagtctagggtaccttagattgtatgggtaaaacatggtttatttaaatcataaataaacagtcttatttccctaaatgcacatacaggcatccacatcaaatgaaatcacatcacatgaattgaacaggcagttactgacttagaactttgcactcacaaaagacacactctcctaaatgtctccatcatactatactttttgtccccaaatgcctaatcactgaagcttcagactttgttgctttgattcccttaggaaaaattcctggtgtttcagaaaaaaagagccatttaactacattagaagttaaccctcctttaaaaatgtg

SEQ ID NO: 20 - DNA, 26803 bp, Homo sapiens
cagttaaggtggggcaggaataaatcacaatggtggaatgtcatcagttaaggcaggaactggccattttcacttcttttgtgattcttcacttgcttcaggccatctggatgtatatgtgcaggtcacagggcatacattggcttagcttgggctcagaggcctgacaaggcacagaaggagctgggatagaggtgcaaagtactcatgctgacctgacatcccatgcccacggcagacatgactacttgatcggacaatactttcttggaatcaaagacacaacttcacagtcctcagcatcatagttcaggcagcctgtatcagtagatcagagtgggcacatggcctggtgctatcactccatcctgtgaggggagatgggattggaatggaggtggaggagtcacaggtggtcctgatatcacaggcctgggagtctgaaagaagtgcagtaggtagtattatggccctcaaagacatctgtgtcctactgtctagagtcaattaaagtgttacctaacatagaaaaaaggattttgcaggtgggattaaactaaggatctcaagatagaaagactctcctggagtatccagttgtgtccaatgtaagaacaagcgttctcaaaatagggacacaggagattgaattgcaaaggagatgtgctgataaacggagaggttggagtgatgccgccatgaggcaaggaatgtgggtggcctctagcagctagcaatgattcggaaatggattctcccccagagtccagaaagatcacagcagtgctgacaccttgatttgagcccagtgtcacctctgtcagacttctgccctatagaactgtaagaggataaatttgtgttttaaggcacaaagtttatggtaatttgttatagcagcaatgggaaactaatacaagaagggttgtgttatcaacagaaatacagcaatcagaagaaagatggttggggagagcagagggtggggtgggaaggtgatggattctgtttgggacattctgggtgtcatatgaatattattggggaactgtccatcaaaagctcagacttcaaagaaagaaaggaaggagcaacaatattttgaaagggagaaagtaggtaatattcaatatgtgttgagtacctacaaggtttttagttctttcaccaagttattttatttaatttttatggcatcaaggggtgttttttttttttcttaaaccaaattttctcagttaagcatcccatgtaagtggccaggggttaagagatgtgactaagactagacagagtgattttcatcattacatggtactatggttctactgaagcactgaggaaggaagtcaagagagttcctgagaaatgtctggagtcttagtaacatgcaaagtgaggcagaggtattgtcagtgttagctggtcactttgaaaggttagaggtaaataaagttcagggcaatggtacttggagaggagtgaatctttggtaacctggaggagatgcttctcagaggaaaatttcttcacagcatgaagtcaccagctctaagactagtgggtgttctgggggatgttagcagtgactcactgactgttggcccagtgaggggagggatgaaaggctgggtagtgggtagagaatctgactcctcctgcccccacatgtctattcctgggccttctcttggtgggggcaaaaggtatgcaaagggatttccgcagtgtctgagtgctcccaggagacggaaaagtaactgatgacttggagttggagtcttgttggctcaggcagctggggcgttttgggatttcaacacctccctttagtttctatgtatggtgctgagcaagtagtcaaagactttggtcttgctttaccccagtagcccacaagcctgagtacatggctaacatttattgggcacttagtgtgtgccaaagagctttatgagacaggttctttttgagtcccattatactgataatgggactgataagaaacagaaggtcagaaaggcccagtaacttgggcaaggtcatgtagctagtaagtggtccagctgaaatttaaaaccaggtttatccaactccaaatcccacatctgatttattttgccatgaattaaaacatagttctgattttgagaaactcccagtcccagtgggaaaacagatggaatcacaaattaccataacacagtgtagtgatgtagatataaaaacaaagacatgggaaccctgaaaggaagttgtaacaccaatagaggaatgcatggaggagatctttcagaggaggtagcctcgtagctgggctcaggggtggatgagtttctggctagaagcgcattgtgggtagagggagaacatatatagaaaggcatgaagatggtggacatgtttggaaagagtgagtactagactgatgaacacgatgagtcaggagcttatgacgtcaggggctactgctagcctagctaatgactgaagattctgtgaaaagaaaaccctaacatttccagctgagtactagggccatggtgattatatatcatctctcatgacaacacaaatgtttgggcttacttatcatcctgctcagtaatcattatgtcactcattaaagatgtatcagggtaaattttaggtgagaattgattagaaatgtaaactctatatatgtagttacaggcttcacagtttgccactcaaacaatatggtcatccaatcatgaggcacaaccttctgctcagaacttttttataattgggagaaagtgacatccgagttccatctcttctgagaactgtgcagctcagaaatcttcttcccttttttgatcccccagttgggtgagatgacattaacagtgtgttataagcacttttcatgtttactaccccatattcaaaattaagcatttcaaacaactgtataattgtctataaatgtagcattattagttaattttccttttaacacattgaggttacctctaatgttttgctatttttaactatgttgaaataatcatgtggtttttattctttgaattattttatattgtaatgttccctgaaatgaaattagttgatcaaaagatgagtaatcttttcatgacttttgatacatgtcactcaatcaccttctggaagagttggaacaagagcctattgctggcatcccatttcatagccatctcaccaatgttggaaaatgggcttttcctattttctgctaattcattagttgttaatggcttattttaactattaatcccttgttattgatgaaagttaagcattttctgtatttttattttctgtctaaattctactttttgcacaatttcctttgctcacttcttcactggaatttagtatttttctttccaatttgtatgactccaaaatcagtgataaaataagcaaagggtctttcttagaggctaaacaagggaatgaataaggaacaagaacagcaaagggatagtgaataaagatacaaaataataacttatttttatttttgaagctttccccaggcagtaattcttgacctttttaagattataaattattttgagatatgcattcttatcctcaaaatgaattagtacataaaatttaaatgggttgatagatcccctgaagtgtatccacaaaatgctctcaggttaagcaacattgttctataataactgctttaaccaaaatgtttaattattgcttgtgtttacctgtcctagcaaagagctaattgttaaattttgtgttagagggtcaatattataaataacttaatgtggcctctctttcctttcctttttttgagagttttgaggctatcactaagtgggctttagagtaccaggtgggaatctgacctcactgctcaaactttcaacttcaggcatgaagtggtcccagtgatgtgggaacctcagagtctaaaacaaaaatagtagactgaggccctcagaaaccagacttatcagattcagaatttaatataactatgtttgaaagatttaaagaaaataaatcaaattaaaaagtgagcaagaagcaagaataacaaatgaactggcatatttgagaaagaattttgagcttttagaaataatacatacacttattgaaataaaaactcaagtcaataggtttaaacagcaaaatgaatatagttaaagaaaactattgtgctgaaagatttaaaaaactattacacagaatgcaaaatgatgaaatagggtaatttaatatatggcagatatgttaagacactatgaggatagtatgagaagacctgatagacatctaatcacagcaccttaaggtgaaaatagagagagtgcaccaatattgaggagttaatgtctgagactattccagaactgataaatagatgaatctacagatctcagaaacacagcttttacaaaggataaatgaagagaaattcaccagagatacattgtaatgaatctgtaaatcaccaaagctaaagatattatttcacaagtggaatgacagctgacttctcaacaacaacgaaagcaaggagacagttgaaagacatcttgaaaatggtgagagaaaaactaactgttaatataaaattgtgtacctatcaaaaatatcttttggccaggcgtggtggctcacgcctataatcctagcactttgggaagccaaggaacgtggatcacttgaggtcaggagtttgagaccgagaccgtcctggccaacatggtgaaaccccatctctactaaaaatacaaaaaaaaaaaaaaaatagccatgtgtggtggtgtgcacctgtaatcccagctacttgggaggctgaggcaggagaatcgcttgaacccaggaggtagaggttgcagtgagctgagatcatgctgctgcactccagtctgggtgacagagtgagactgcctcaaaaccaaaccaaaccaaaccaaaccaatctttcaagaagtacaccataaagacatttccggataaacagtgaatgagattacttcctaaacgaatatgtaaggatgtttctttttaaaattttttttgggtgtattcatcacctcaagcatttattcttttgtgttgttacaactgataagaatatctaaggatgtttcaaaaggaagaaaaatgatccctaaagtctggtatattagtttcttattagttgctctaagaaattactgcaaacttagtggctttaaaaaacacgaaattatctttcagttctgtaggtcagaaatttaacctcctgatttctggtcagaagtcttactgggctaaaatcagggtatcagcagggctgctggaggctctggagatgatgtttctctaatttctagaggcatttgcattccttagctagtggcttcttcccacatcttcaaagctaacagtggcagtcgagtccttctcttatcttttttttttggggggggttataaattttttttattattattatactttaagttttagggtacatgtgcacaacgtgcaggtttgttacatatgtatacatgtgccacattggtgtgctgcacccattaactcatcatttagcattaggtatatctcctaatgctatccgtcccccctcccccaccccacaacagtccccagtgtgtgatgttccccttcccttctcttatcttatcactctgacctcttctgcctcctttctctacttttaaggacccttgtgattagattgggtccacctaaataatccaggataatctctttattttaaggttagctgattagcaacctcaattccatctgtaaccttaatttcttttttgccatgtaacctaacatagtcacaggcccaagggaataataggatgtgggaattgcgggtggtggagtaggggcattattctgcttaccacaggggaccttggatgtcagtaaaaaatggtgaggaagaaaacaggaaacgtagaataatctaaacaaatctttgaaaaataagttgaaatgtggggttagaaaaagggcagaactaaaatgttaagacaaattaaaatgttaagcctataagttgagagggagatgatcaaggttaaaaatactcataaatcatatttttttgggtagggggttagatatttattaattttagaccctgagaagtaaaatagtcatgacaaaaatttaatagtaaccactaaaacaagagaaacagagtatataacttctaaatcaatatgggaaggggaatggaataagaaaacaatagcaaccaccaacaccccacccaaaataaataataaggtgagagagaaaaagaagcattgaaaaggggctaaaataaaataaaaaattaagtcatgcccgtaatcccagcactttgagaggccaagatgggtggatcacctgaggtcaggagttcgagaccagcctgaccaacatggggaaaccccatctctactaaaaattcaaaattagctgggtgtgggggtgcatgcctgtaatcccagctactctggaggctgaggcaggagaatcgcttgaacccaggaggcagaggttgtggtgagcagagattgtgccattgcattccagcctgggcagcaagagcgaaacgccatctaaaaaaaaaaaaaaaaaaattaagatagtaaaacaaatccaaatacattaaagattacaaaaaatgaaaatgaactaaacttcctagttgaaagacatattgtcagattggattttaaaatctggcaatgatatttccaggacacagtcctaaaatattaaacacagaaaagttgaaagtaaagggatggaagaacacagtcaaactaactagaagagagctgggttcacccttttatatcagagcagaatttcactgagaaaacactaacaggaagggggaaaggcacaacatagtgatgaagcacttaattctcaacaaatgtatgacacttctaaactattatgactgcaaaaaaaaaaaaaacctcagcatatataaaattttggaagagccatggctatcagctgacatgcacttaccatatttgcattgtcctactacaaactttacccatatgaccaaggtgctgtcttcatccccattttacagatggggaaatttccccatagagaaaaagatttgggccatgccttggtttcttcttgactctgcttcctgctgattgatcctcacacctcacctggagacctacttcacattatccatcaggatgagaactggtgtgcctttaccaaaggaccacagtcaccttcaaaacgtgtttagatagatctggatggagacttatgtggttgcagatgaaaaaaaagtccccatggtatatctgactccatgtcattcactgcatgaacactcacacacatgcacacgtacacaggcaaacacaatcctgttctggtccggcagtagtgccaacactcaaatcccaggtcctactctgaagcctttgaggaaaccattgtcattctggggtttatgggaatatttcttcttggtgccccttgttcctcacagaagctttttttctgtgctgtgggcttgctatcctagctttccaagctatcctagttttgcaaatttctctgatcaatcacatcaggttcttggatcatcccaaaattaaagaggtacgttttgctgcaagagacaaagacattcacctctcacacagtttgaattcctgggtagaaacagatttcaatgctggccagcctctgtagctcccagtgccccctcaattatgactcccgaggcattggagcaggatcctcaccttgcgcaaagataattaggtgtgctgaagaaagccagacactgctctttcttagctctgcatccttaaaaagttaccactactccttctctttgaatctttgacttgtcaatggtaaagtgcctatgattcttaaagggataaaaacgcaacctatataaagcacctggcatagtgcctggcacaggtgggtgtttaacaaatgttaactcctttctatcccactgtgggtgtccatatcctcttgggtaggctgcctctggtttccattgtgtcatcagagccatactaaatcgatgtgttggacatggatcccaagaactaatttctggaatgagttatgcctaccaacttccctgatacttacttctgtctctccatttatcaaatggaaatgtttgcatttggcctctgccagttggagtaaccaaaaggcttagaggttttggagaggtcctacactgccatctgtttgaccacatactgcctttcacgtgtaataagcattgtttcttacatttgtctaggaattagcagttcacaaagcacattcgcatataagggcttgttttgaattgatcttggcagcaattctatgagacaagtaaaaggtaggtcaagcattataatcctcattttaaatctgggaaaactgaatctcaaaaaggttgaaagacttgtctaggggacagtgtgtgggtaaatgagaagttaagatttgctgaactggcatttcctgactacatatctagtgtttatttatggagaaggcactacggtggccaagtggctcagagtcacacagctctgtgcctcagtttatttgtctgtaaaatgaagataataatatattctgaatactgttgtggaatttcattgagatagttcacataatggcatggatactgtagtacaccgcctagattcacaaccccacgactatccatgagaatggcccatagctcaagaggtcacattctttccccaggtgaagcccgcatccaatgactgctcagtgtgggtatataaaggcctggctcccttgccagtgccaccctacctcctggcgaatggactgaggcttgcattatgactgcattgcagctcaactgttctttccattcagtctttcctttacactcacacaggtgaggacccagccattaaatgcctcacatgatgacctctattgcatgctaggcttcgtgtgcacacacaaaaaccatcctctatcagtcaggccccttacttgcagaggcaaagaggccagtctgggttagatgtgcaccctgtttttacaacagaacgagacaaacaggtcctccttaggtgtaagttcatggccttggccccacccctgaaactcagccatctgagacagttttaggactgaggcaaccccagactttgggttgttgtttgctgggcacagcctccttttgccaatgttgcaatcctttgtaagagaccacaggttgatcacccgttcctgttactgagcacagagaggtttgtaggccagtctctccaggaattctgacgcactgcaaaatcccatggtctgaatgcttctaccttccctgtgaaagcccctggcctcagaaaaggaagctggtttaagtgaccaacatttggggtggagcttccgagggcccagccaccgtgttacatgcaacaatcaacagagatattctttggctagagttgtttttctgggtataggaccctataattaaaatcagctctccaacttcccttcctccaaaaagtatacaatgtaaggaggaaaatgcaaattgaaaagttgctagcccttcccgccagaatgccaccccaagcctcccctgcaggaagttctggagtccccaactctgccccaagcctgaggcccttgataaggtaaagggatgtgagtgtggaggccggagcccccctcgccctgtaggctgctccccttgcttttccctttgaatgttacagtttagttctgtgacttacttataattgcctgaattccccgcccacgctttctcttactttggggcttctcaccgttcctcttcctccatcttcctcctctgaccccactcccaagcctgaatggggtgttcctcttccgtgctcccacaaaaccctgtgcctctttcatcgttgcatatattatgctgtaatgtagttttctggaggtgtgaagactatgaatcctatgaagacaaatacacacctaccttgctgaccgttgtatcctcagaatctaatactgcacttggcacacagtggttgggagtaaatattcatgaggcaaacacacaggaaggactcttttgttatggttgtttgttgttgttgcaagtaacataaccccaccttgatctagctgactgacggctctaccaccttgtcttttgcagcacaagaggaataggaactgcacctcttccttcagtttcagcttgaataatatcaggaagattcgtatcggtctgagttgggtcacgtacccgacgtgctatagctgaggatggggtaagctgattggagtttgcaacactgttcacatagccaagatatggaaagaacctaaatgtcaactggtggatgaatggataaagaaattgtggtatatacatacactggaatattattcaaccttaaaaagaaggaaatcctaacatttgtgacaacatggatggacctggagggaattatgctgagtgaaataagacagacacaaaaagacatttcttgcaggagctcacttatatgtggaatctaaaatagtcaagcttaaagaagagagtagactactggttgtcaggagcaggagaaaagtggaaatgaagaggtgatagttaaagggtacaaagtttcagttatacaagataaataagttctggaggtttactattaatatatcacatagtacctataagtaacaatactgtattgtatacttaaaattgctaagagggtatatcttatatgttcttaccaataataataataatggtaataattaaggggcaggaggacacttcaaaaggtgatggatatgtttatggccttgatggtggtgatggtttcatgagagtatacttatccccaaactaattgagatgtaaatattaaatatgtacagctttttgtatgtcaatcgtacctcagtaaagtagtttaaaaatggttggactgagaaaaggaggagctgctcagcaacatgaggctgggtgctgggcagacaaaacctcacacatgcattactgaacccacggactcatgtctgtgagctttgtggctgtggatgcaccatgccaatgtagtcaaggattcttcaatgtgtaccttactggattagttccctctgtttatttgtattgactcctcagttcccttatgggttgcttgttggctcttgtggaattatttaagtaaggctttggttgcaggagtcagacatgcttaagctggttttggctgtaatggggaatttgtgagatgtgacacagtgacaggaagtgcagccagacgttgtgagaggcagtaactgggaataggaaagttatgagaagttaaggcagtagtaattgtttctctatcgaaggccataatgttatcattcctgcctctatctgtttgcttgttcttctctctcagcagaatggtcttctctgcttctctgtgcacctgcagaaggtgaccaccctaaggcttatggattcaggagtcctcagtttgagagcagttaccaaatgcctcgcccctgtgaactctagtcccagtttcttattcctggtactggcttagtttgaggcagctgcccaccgtaagtccagtgagccatggcctggggacaaggtcaggtacatgtgtaatcagctgggtctatgagttgtggtggtggcgatggaggtagctcccagaaaaatggattacaggttaagaagagtctatatatcttgaccacatttgatgtgacttggaagtttcaatgtgtgaccacttacaaagttatgatcaggtgtctcatttatttatggtgatgtatgagtccgtgtgtgagtgtgtgtgtgtctgtgtttgtgtgtgtgtgtgagagagagagagagaatgagaatatgagtggtggtttcccatttatttttctatgggccaaatcctgggctatgagctggagatataagagtaaacaaaatagacacggtgcttgctgtgacctgccctgggagacagatattacacggaggatcacataaatgcagagtctgagctgaggtcttaagggtgaggataagtaactagtcagtggagcaggggagggaagggtgttccatgcctgtgtcaaggtcctgaggtgagagaaagaggtgaatttgaggaaccaaaaggagttcagggaacaagaggggctgtttcacaagctgagtctggaagctgagcaggctgagcagattcttaggaactctgcaaaaacttaagggcttgtctatgaccgtaaacaactacggtcgtagataaacaagttggcaaacaactcaaggatttacagtcatcagaattgtaaaactgatcccatgtattttcaaacctcaaatcccttgctctgaccttgtgtgtctaagctagaaggaagcaggatgcacctctcccctggctggaatgaagggattcacccaagctctcagtcttctcacggcatccagggcccccctgcttgtgtgtggtctagatttccattcccatagtaggaattcctttgggagccttggggtctctcctgctagagggcttcacctgtgactgtctcaattcaagggaggggttctaataacattaaacctcaatatcttgctcttccattcctgatgcctccctttccttctacccttcccctacctccttctttcctatgccacaggctggcaggttagtgccagagcaagtggccagtcaccatcattggggttgtggatcctcagggttcttcagaagccccttcaccatgatcaagagtctccagtcactcagaattccacggttcccaaatgccagctctcccactactcccagcgttctccatctctgggatgttgggctccaggcttctcagatgcactgagtaccctaggctaagccactgatccatcagaacttcatagcctgagaggagagggagacaggcttgcaaaggagagttctgactagacactggggtgctacagatgcccgtaagttgtccctttaccctcgatgtccccagtgttgggaccacctgggaatgcccagccttgtgtgctgattgacttgtagtcccctggccctgactggaagcctagttttctctctcatgaccagctaggcccctagctccccagggaagaaatccaatctatttcctctgatagtaatggctaatacttaaataatgccaaccacatgccaagcactttacagttgttagcccagtcttcacaagcaccttgtgaggtgggcaagagtcttatcttactctcattttatagatgtggcccaggatcccacagctatagttcatggtgctgggatttgaacctctggccaccagagcccaccttaatgtgtcctcctcctgttgtcataacagaaaagtacaacaccatgatgacacatcaggctatcctggcaggttcccaggctgccccaatgcccaactttctaggtttacaaagttgacatttacgaagtttccaggtttacaaatctagtttctgattctttagtcagcaggaatttctctacaaaagctgcttcgaaaatttccagccaaaccttacacaccttggcattacatcttggtgagccaaggcggaagagaacaggaagtgaaggccccatgggaagtccctgcggtcgggagcacccaggcggggcggggggtggggggctttcctgtggccggctccctgcccctcccacccccattcaggccctgtgagttgaatgaagagaccctgggaatgagtccaggtctgcagggttagaggaaattgaaggcccttaccagatccctgttgagaagtttatgaattatgagcccttctgcaaatgagagggttcttccctgtcaggagggacagattgtaggtggcaagattggtggcagccagtaggctggtctgctccttcctctctatttcatatgtgtatgaaggcattacctgcagcaagggcctgtgtaaatgcatgtgatttacagagcattttatgtactgcgtgtcattcatgcttccggtgagccctaagtctaagatagggcagatagcatcaggtccattttgcagctgtcaaaatgaggtctgaagggcagaagtggtgtgcccacacacacacaactggttggctgcagacctggggactagacccgggacttcgtcctgcccaggggtctcttgccactgctccccatcaacttggatggctttaagcatttgtgagttgtctgctccctgatggcagaatgcagagacatgaagctacaagcaggttcgctcccaacggcaaaaaggaggaggggtgttcagaacatcaggtgcttctagagaaagcagggagagagtatctggccttgtggacaatgtcacggcagaggccaggtatagggcatgggggtaactggaagcgggatggaccctgttattccctaagacatggcttccacgtagtgctcaaacaaggcctttgcccttgctgttccctccacctggaatattcttccccttccttgacattgctcaggtctccactcttatgtcaccctctcagagagggcttccctggccactttccctaaaatagccacccactcctaggtccctcaaaagcatatcctgctttggattttccctatagcaatatgccctatgaagttattttatttgctaacttgtttcttgtctgttttcctttgttagagcgttggggaccttgtctggcttgttcccaatgcctggaagagtgcctggcacacaggattaagccaacacatatgttttgaatgaatgtgtgcacacatgcatgagctggcggcagtcggggttggggtaagcacgaaggcccagctcagttctctgcatgtgacctcccatcttacgcagataagaaccagtttggtttctgctagcctgagtcaccctcctggaaactgggcctgcttggcatcaagtcagccatcagccggcccatctcctcatgctggccaaccctctgtgagtgtgtgggaggggaggctgggctcctccttgtactctctgaggtgctctggaaggaggggcagctccaccctgggagggactgtggcccaggtactgcccgggtgctactttatgggcagcagctcagttgagttagagtctggaagacctcagaagacctcctgtcctatgaggccctccccatggctttaggtaagctccttccactctcattttttcacctgagaaatgagagaggaaaatgtctacaattggtgtttatcaaatgctttcaggctctggtgagcaagcgtccaggaaaatgtcaagcgcatggagctccaggcctgtctgggggatctgggcacggggaggcatccatgggagaccatgcaggcactctgaggcaggggctgcaagcctagtgcctgctggggcagcaggtgaacagagaggtgtaactgctgtgacagaagtcatggagtccttggagtgtgagggtcattttccactgttgatagaatagggaaattggtgaaatagccctgttaaatgagagaaagaacagtgtgagctcaatgagaaatactaatagaatgtggcactgagccacaaggtctgaggcttgattgataaggaagggtggggactgtggagaattaagggcttggcacaggtcagttccaccagttgtcacaagagaatgcaggctcaggtggccagaacttctcgcttttccagaagagtccgatattctgatttcattatatatagtattctgattaaaccagacaataaagcaagcagataaaatatttaaagtataagctgccagtttgcaacctccggttaggatttgtgtggggcaaagaaaaaaactctcaggatcattggtatgtagactctaattttaagtttctaatttaaaattggcccctgaggctgggcgtggtggctcacacctgtaatcccagcattttgggaggccaaggtgggtggatctcttgaggtcaagagttcaaggcctgcctggccaacatggtgaaaccctgtctctattaaaaatacaaaaattagctgggcatggtggtgcatgtctgcaatcttagctacttgggtagctaaggcaggagaattgctggaacccgggaggtagaggttgcagtgaatggagatcacaccactgcactccagtctgggcaatagagagagacgctctctctaaaaaaaaatatgtaaagataaataaaatgaaataaaataggcctctaatgagcaggccattctcctttctgggtcttactttccttgcactcctttctgggtgttaagaggaggtctagaggaagctggacaactcttagcttgtagtaagcacagtggaagtatcagctcttaatgggtcatggacacgttacaagctaggcgccgtgctgagcactttacatggtttatcccactgaaccctctcaataaccctatgaggaagggctattattgctcacattttcagaagaggaaatggatatagagagattagataatttgcccatggccagacagctagtataagaggaggaggtggattgactgcagacattctgtcttcaaaccactacactatgctatggaggcacagagacttaatgaaatcatggagaggggaattgctttgtcaaccacaagcagttattccgggggcagcagatcctcccctgtcccccagtgggtacaatggtccctggtgggttgtgctacaatgttagcccatggtcttatgtgtttttcaaatgtgtaaagtaggatgctggaaccactcttagaaccagataccaatacattgtgaagaaataaatctctgtgcttaaaactggttcatcccaaaatattttgaactgacacacaataggtgctaaataaatgtgtgttaacttgaattggattgaattcgggaaaaaagtgcaataagcttagtgaagacaccatgttccctgggtagaggaaccacattctccatctaaggccaggagtatgggaggtatcaatgtttgcccagcacagaacagggtgccaagaagagaaaagttgacggggtgcatactctgactggaaactggaagggtgagaacagagggtaaaggatagagatggaaccatgtgcatacactttgtgttaccttggacaagtcattcatttctctggacctctgctttctctctacacaatggggtcccaccacttcccttacagctgacttgtatgaagaaggaggtggaggaggaggagaaggtgaagacaatgctgactcaaagggtaaattatttttaggatccaagtttgaaaacaattttaggctactagatatgaacaacatcttgattatgtagttgaaggaaattaaagatgaatggtttaattaaaaattaatcagaatgaaaacgattgattactaatatatctgcaatggtttattttcctgagtggcagactcactaaggtttttgaatactcctgtgtgattgctctatgtatgtatgtatgtatgtatgtatgcatgtatctatctatctgttgtctaataaaatggatcacatctctgctaataaaaacactacactggcagggtacaattataatcattaactgtgcctggaatttgcagcagcagccaccagaggtaccagtgccctttaagggttcataatttagaataatccaattatctgagtttttcagggactgaggggtttggcaaggtgtagaactttcagtaataaagtcaagaaagtcctggacaaaccaaggtagttggtcactctagtccataaccaggtaaagagctttccctgtaacctgtgtaaggttttagaatcatttctttccttattaccaaaaatcctccccaaattttcaagaaattatgaactaaatagttactctatgagataggagttcagcccaaaagaaacaccataagaacaaatataattcttgcttatgttaaccatgcaatgaagcagagagaaaaagtcagtggcctctttaggaggactgtagtgtgggaagaaataactaaactgggtttcaatcctggcctggccaggatctggagcaagtgagttaatctttctaagccttgagtagtttcttcttcttcttcttcttcttcctcccccttctcctcttcttcttcctcctccttctcctcttcttcttcttcttcttcttcctcttcttcttcttcctcctcctcctcctcctcttcttcttcttcctcttcctcttcctcttcctcttcttcctcttcctcttattcttcttcgtcgtcttcgtcttctttttattttcaaagtgaaagcaagtttattaagaaagtaaaggaataaaagaatggccactccatagacagagtagcctgaaccttgagttcttctataaagtcactatgaatttatactcattttgaaagtgggtgtcaatatgtctgtccactttgcacagctgttatgtggacaaaaggagatctgtgtgaaagtgtaacacagagcctaaactataacaggtaagcaacacagttgtccccttccccatggtgtctgttcttctccatttcctcctgtctgcagggggattataaaactaatcatcaaagccaagaaggcaagagcaagcatgtaccgctgaaaacacaagataactgcataagtaatgactttcagtgcagattcatagctaacccataaactgctggggcaaaaatcatcttggaaggctctgaacctcagaaaggattcacagtaagttaaccatgtagatctgagaggagagtagcttcttgtagataacagttggattatataccatgtcctgatccccttcatcatccaggagagcagaggtggtcaccctgatagcagcaagcctgggggctgcagcttggtgggtagaggtactcaggggtacagatgtctccaaacctgtcctgctgccttagggagcttctaataagttgatggatttggttaaaattaacttggctacttggcaggactgggtcagtgaggaccaacaaaaagaagacatcagattataccctgggggtttgtatttcttgtgtttctttctcttctttgtactaaaatatttacccatgactgggaaagagcaactggagtctttgtagcattatcttagcaaaaatttacaaagtttggaaaacaatattgcccatattgtgtggtgtgtcctgtgacactcaggattcaagtgttggccgaagccactaaatgtgagatgaagccattacaaggcagtgtgcacatctgtccacccaagctggatgccaacatttcacaaatagtgcttgcgtgacacaaatgcagttccaggaggcccaaatgaaaatgtttgtactgaaatttgttaaagcttcccgacaaactagatttatcagtaaggattgttttctgcaagggggatgaaacttgtggggtgagccatttgggctgaggaggagggaggttggagctgagaaatgtggagacaatttccctttagaaggactgaatctccctgcctctctggggtgcggcagccagcaggatccaatggtgtatatgtctccccagctccccattcagtgatatcatgtcagtagcttgaaattatccgtggtgggagtattatgtcatggaaattggcaaatggaaacttttattggagattcaattgttaaacttttaccagcacaacactgccctgccttcagagtcaatgaccctatccaagtttaatccatctgtccactgtctccaacacgatctttataaaacacacctgacaacattacccttttattcagttttttaaaagataagtttccagctcatcggggtggctttaaaggccatttctcctctggacctcacccaacttttcaaatcacttttcctacccctacctctaaatgctactcaaactccagccatcctgaataataagacttttgaaaagtagattatgggctgggcacagtggctcacacctgtaatcccagcactttgggaggccaagatgggtggatcacctgaggtcgggagttcgagaccagcctgactaacatagtgaaaccctgtctctactaaaaatacaaaattagttgggggtggtggcacaagcctgtaatcccagctactcaggaggttgaggcaggggaattgcttgaacctgggaggcggaggttgcggtgagcctagattgctccactgcactccagcctgggcaacaagagcgaaactccatctcaaaaaaataaataaataaataaagtagattacatcagatacctctggcctaggttgtttatgaccaactctcctgctgagaataactagaaaagctagacaaaacatatttccaaaagatctctttggaggcatcagagaatggccaaggctgtaaggaactgcctgagcccagagaggtggagcccagcactggtgccctttactcctggggacatgtgctggtttcaaaaacttcagctgagcttttgagcattcatggaacttggtgggggagatgaaatttgtaccttaaatcctgcctacagggagggtccctgataatccccacccaatttggaaatctgggtcagccttcacaggtactgaagccctcctctgaatgatctcaagtcctgctagggtagaggttacctgcttttgaaaggctcctggcctacctgtgcagcaggagcaaaagtgaaccatctcagggtacagataacaatcatccagagccttgaatgacctctactgtgcttaatatatagtattcagcagtcagtaaaaaggatttaggcacatgcaagatgacctgtgtatcagggagaaataggcaataaattgagatccagcagggatttgaatcatggatttgaatcaggggcagccttcgaaagaactatggagaatatactcagatttaaaacataagattggaatttttggcagagaactaacaactgtacaaaaaaggaaccaaatggaaatcctagaactgaaagatgcaattaaccgatgttgagaaatagccaacatctattgaacacttcccatgtggacagctgtgctaaacactttacaggcatcaacataagatgtgtccccttacagcagtgcagtgtccctcctaagacatggacagcctggtttccctatctctctgcttcatcaaaacccctttacgtggggcttagacactcctgttgtctctagtgtctagtagcacagggctcagcacatggaagccactagatacaatttgatgaccaggacctccgatgaaagccatgggtgctgattgggaaggcattgtcttttatgtgctatggtcttaaagcttcatccaggaagcagaactcggggggtgctgaggacccagaaccgagaataagattagtcagagatttcctgtgggcagaaatcataaggacgccaactgtttgggtgagataagacgaaaccaagagtggacttgtggccagaagcgtgaggaagagggagagagcttcccttgtcccctttcttcctctccctaagccacagtgattgacagccccccccctttggagtcagagcaggcttgagactggactgggaaaggagggtgggtcaggatacagagcaggaaggctgggagtgcagggcaggagcaaggggctggggcattcattgtgcctgatctctcccactttacctggggtaaagaagcatatgcaaaagccacggtgtgagtatttcccaagtgccagggtcagggcatgattcatcacgtgcagcatttcattcaatccttatagtaaccgatgatgtggcttctattattagctctatcagataatgaaactgagaccaagacaggctctgcacattgtgtggggtaatgacacagggggattcagacctagactccataactcctgccccagggaccacccccaccctcaccctgtgcatgtcgacaaaggacagactgggccacttctcaggacacagcggggaaatgacacagagcagggaggttccaggagccccgagcgtcttttctccaggagaatactctctgaattcagactggggtcagagaaacatttacccaggagccgcagtgtgggtggggctttttacttgaaacgctgtctgaaggcagtggccaggatggaactctccaccctaccttggcaagccacttctcttctgcaatctgtaaggacattgttgagagaattatggtcttccaattccggagggttgaagaaagacaaataggagagaacctatcatagtcaggtgctagctgccttctctttcagagagtgtgagaataaagtgatacacttgattattagcaaatactttggaaattttaaacgctaatattcaacacactctggaagaggcaaataagtagacaggttcatatacatcatctccttcagctagtcctcacaaaaacaaacaaatgaataaacaaaattcttctttggccctcataggaagacactgtttcttgaacgtgtttcaaaaaggatgggtgactcactcaaggtcacactgtttatgaggacagtacaggaatacagacatgccattttgcctgaaaaaatccatcacccagggaggtgacacaattttgcagaaatgttctatttcctctgaaggatacattctttaaacctttgggaaattcattcatagtcttcctcctttgaaggattaactctctggacacaaagtgtttgattctgatttgttggttggaagatgtgttggttgagagaaagattctgatttgttggttgaaaatagactcatcaagatcaactgctgtagtagtaaatattttgacattttgtctgtattcctgtgctgccctcacaagctgcatcaccttgagtgagtcattcatacttttttgtttgtttttgttttggagatggagtcttactctgttgcctaggctggagtgcggtggcgtgatcttggctcactgcgacctccatctcctgggttcaagtgatcctcctgcctcagcctcccgagtagctgggattacaggcacatgccaccatccctgctaatttttgcattttcagtagagacggagtttcaccatgttggtcaggttggtcttgaactcctgacctcaggtgatccgcccacctcagcctccccaagtgctgggattacaggtgtgagccaccgtgcccagcccagccatcatttttgaaacacgtttgagaaacagtgtcttcctttgagggccaaggagacattttttttgtttatttgtttgtttttgtgaggactagctgaagggggtgatgtatattaacctgcctacttatttgcctcttcccagagtgtgatgaatattagggtttaaagtttctgaagcatttgttaataaagcccggggctggaggtcagaagacctggatttctctgcatacttttgccatcagcaagctgtgtgaccttggacagatcccttttttgtctaaatctttctgagtcttcttgaaaacaatgccaggttgggacaggatgattgccaagctcccgtccagctctaaaacactgcaacgtatgcttctgcaccagcactgtccatcctgtagatcatgcagaaattctcttcaactttttcctacccataaaataggagcatgcttacctttttcctaatgttccaggccccgggtctagaatattgtaagtaaggaagttaatgtgtatcagagcccattatgggccagaagttctcctcttccttcctacacctgcttcctccctccctccctccctctttcccttccttccttccatccatttgtgaagaagacatgatcaccctcattctgagagtgaagagacagaggctcaactaatgaaatgatttgttcaaggtcacacgggtggcacaaggcaagtggcagaggttgaatttagacccattcctgtccaaatgctgagtttatgtcatcgtcccgagaccataactttaaagatgtaagatagtgggaaaagagttgatttcaaagcacctctcagaaggactcactttacatcaggggtcagcagactcaggccaaatccggtccattccccgcttttgcaaagaaagttgtagtggaacacagctaggcttattgatttatggattgccaacgtccttttgtgaaacagacagctgagctgagtaatcgtggcgcacaaaacctaaaatatttactatctcgtcctttacagaatgtttgccaatctatggtccggagtccaaggctgtccatttttcaaagaacacaaagtgacatgagactgtcccatgtgcagggagccctatcattttattatgaaaaaacggcctttctgctcaaatctgttttttaaaaagtcaacaaacagactctgggtacctgtcaggaacagtagggagtttggtttccattgtgctcttcttcccaggaactcaatgaaggggaaatagaaatcttaattttggggaaattgcacaggggaaaaaggggagggaatcagttacaacactccattgcgacacttagtggggttgaaagtgacaacagcaagggtttctctttttggaaatgcgaggagggtatttccgcttctcgcagtggggcagggtggcagacgcctagcttgggtgagtgactatttctttataaaccacaactctgggcccgcaatggcagtccactgccttgctgcagtcacagaatggaaatctgcagaggcctccgcagtcacctaatcactctcctcctcttcctgttccattcagagacgatctgccgaccctctgggagaaaatccagcaagatgcaagccttcaggtaaggctaccccaaggaggagaaggtgagggtggatcagctggagactggaaacatatcacagctgccaggggctgccaggccccagagggcctgagaactgggtttgggctggagaggatgtccattattcaagaaagaggctgttacatgcatgggcttcaggacttgtgtttcaaaatatcccagatgtggatagtgcgaccggagggctgtcttactttcccagagactcaggaacccagtgagtaatagatgcatgccaaggagtgggactgcgattcaggcctagttgaatgtgctgacagagaagcagagaggggcaccaggggcacagcccgaaggcccagactgatatgggcaaggcctgtctgtgctgacatgtcggagggtcccactctccagggaccttggtttccccgtctgtgacatctgtgacatgagagtcacgataactccttgtgtgccttacagggttgttgtgaaaattaaatgcacagataatagcgtaacagtattccgtgcattgtaaagagcctgaaaaccattatgatttgaaaatggaatcggctttgtgagaccatcactattgtaaagatgtgatgctgatagaaatgacaggactgcttgtgcatgccctctgcagtgtgacattccagcagtgaaatcatgttggggtgacttctcccccactctgacctttatgtttgtctgggccgaggctgcaagtcgggctctgtgggtgtatgagtgacaagtctctcccttccagatatggggactgtctgcttccctaggttgcctctccctgctctgatcagctagaagctccaggagatcctcctggaggccccagcaggtgatgtttatccctccagactgaggctaaatctagaaactaggataatcacaaacaggccaatgctgccatatgcaaagcactttggtttgcctggccacccctcgtcgagcatgtgggctcttcagagccacctgatgaggtgggtacagttagccacacttcacaggtgaagaggtgaggcacaggtcccaggtcaggctggccggagctctgtttattacgtctcacagctttgagtcctgctctcaaccagagaggccctttaccaagaagaaaggattgggacccagaatcaggtcactggctgaggtagagaggaagccgggttgttcccaagggtagctgctcctgcaggactctgagcaggtcaccagctaatggaggaaaggctctagggaaagacccttctggtctcagactcagagcgagttagctgcaaggtgttccgtctcttgaaacttctacctaggtgctatggtagccactagtctcaggtggctatttaaatttatacttaaatgaatgaaaatagaagaaaatttaaaatccagacccttggtcacactatccacatttaaagaggtcaatagccacatgtggttagtggccaccctattgggcagtgcagctacagaacatttttgcatcccagaaagttcttttggatgttgctgctctacagcatgctttgctgaaacagaagtgccttccctgggaatctcagatgggaagcaagtaaggaggggagtcaaatgtgggctcactgctcaccagctgtgagggttgggcctgcctcttaaccattgtcagcctcagtcttctcatccatgcatgccgtgggtatactaaaatactatacccctggaagagctggatgcaaatttgacaagttctgggggacacaggaaggtgccaagcacaaggctgggcacatggtggctgtgcactacagctgagtccttttccttttcagaatctgggatgttaacc

SEQ ID NO: 21 - protein, 177 aa, Homo sapiens
MEICRGLRSHLITLLLFLFHSETICRPSGRKSSKMQAFRIWDVNQKTFYLRNNQLVAGYLQGPNVNLEEKIDVVPIEPHALFLGIHGGKMCLSCVKSGDETRLQLEAVNITDLSENRKQDKRFAFIRSDSGPTTSFESAACPGWFLCTAMEADQPVSLTNMPDEGVMVTKFYFQEDE

SEQ ID NO: 22 - protein, 159 aa, Homo sapiens
MALETICRPSGRKSSKMQAFRIWDVNQKTFYLRNNQLVAGYLQGPNVNLEEKIDVVPIEPHALFLGIHGGKMCLSCVKSGDETRLQLEAVNITDLSENRKQDKRFAFIRSDSGPTTSFESAACPGWFLCTAMEADQPVSLTNMPDEGVMVTKFYFQEDE

SEQ ID NO: 23 - protein, 180 aa, Homo sapiens
MALADLYEEGGGGGGEGEDNADSKETICRPSGRKSSKMQAFRIWDVNQKTFYLRNNQLVAGYLQGPNVNLEEKIDVVPIEPHALFLGIHGGKMCLSCVKSGDETRLQLEAVNITDLSENRKQDKRFAFIRSDSGPTTSFESAACPGWFLCTAMEADQPVSLTNMPDEGVMVTKFYFQEDE

SEQ ID NO: 24 - protein, 143 aa, Homo sapiens
MQAFRIWDVNQKTFYLRNNQLVAGYLQGPNVNLEEKIDVVPIEPHALFLGIHGGKMCLSCVKSGDETRLQLEAVNITDLSENRKQDKRFAFIRSDSGPTTSFESAACPGWFLCTAMEADQPVSLTNMPDEGVMVTKFYFQEDE

SEQ ID NO: 25 - DNA, 3804 bp, Homo sapiens
taatttcagtgaaattatataacttggttacatttaggttacttattacaaatgaaaataaatatactaacagaagctgcctcatatgcaaatgagtaacatgttagagactaaaatacacaaaaaaatgcatgtgctttagctcatataaacaatatacaggacaacttaccgggtagcataaacaaccaacaacggactatcaaaaggaacctcgtcatctagtaactttaaccttgttggtagatctcctttttccatctccatatacacaggattggaacttgccatttctgaaatataaagcatatccttttccaaactttatctcttaggcggaaatattcaatttatgaacatgttcattcagcaatcattagtcacgtacctactgtgtggacctattatgtgcaaggcccaatattaagcattacaagagaaacaaataaaagtacaagagatgtaatttctacttttaagaaccttaaaatctaattgggaggcaaagcatattaaaagttttaaataagacgaaggaacatataattaatacatcagtgactattactcttaaaataatgagtatctaggcctatatatagcaactgtccatataagcacacatcaaaaaccaatatacatagctatcatcaatgccaagttgctcagttttttctagaactagtattcctactccatcttttagaattaaattcaatgaaattaattttaaaatatttgacctttttttaaagttaccagtatagcaaatactcattctctgaagaacagaagatttgactttttggaatagccaaaagtcacttaaaatcaagtctggtgaaaggagtgatgatctaaaactatttgtggtttaaaaaaaaaaagtatgaatctaaagtaaagtgggtttttttccaagtagttttcttttttagttttttagaaacagggtctcattctgttgcccaggctggagtgcagtggtgatcactgcaaccttgaactcctggctgtgtgtgtgtgtgtgtgtgtgtgcagcgacggggtcttcctacgttgcctagctgcagtgcctgtgtgcacacatgcgcacatgcgtgtgtggagagacagggtcttgctacgttgcctagctgcaatacctgggtgtgtgcatgtgtgtgtgtgtagagacaaggtcttgaaacgttgtctaggctggcatgtgtgtgtgtgtttatatgtatgtgtgtgtagacagggtcttgctacattgcataggctggtgtgtgtgtttttgtgtgtgtagagacggggtcttgctacgttgcctaagctgggcaagtatttttcaactgcctctgaagacaaatcccaaataacagttccaaaagctgtttcccataattatcacatcattagaagggtgaggcctactcaccaggttctaagagccaacattcattttctgatacatgcttttttaaaaaagtcattttttccccagtctcattgtttcccatttgactgtgtcaggcaataagtactttaaaggaattcagaggaggaggccattcagaggtttggggaagcctgatgactgcgcgggagctaaaccagacatatccacctaaattcaagtaagcagccatatcactcaaattgcccaccatgcttcctctagccagcactggtagtaacaactatcactctggctgatggagactcttttctgctcttctgtgactgggtatgatcacataatagagacagatacagtaaatttccaatgagtaataatgtcacacatttgaacttacctgaggagaaatagcttgtttcttatttcacacaaaagacaatctacctcaactcagaaaaaaaaaaattattatgcttttaactgctatatttgaattaaagcagatctgtaactatagatccatgtttctagaaagctaaaatatctttaagtaagatgacataaaaatgtatctctattcacttttggtaatgaatgaaaagttgcttaaagtctaaagtattagaaatatggcatctgttattcaagtaggatttggaattaagaaaattcacttcttcaaaaacatgggactatggctgcagaaagggcaatgcatatagtttttagggtatgatagctggtttctattatatgtcaggatgacatatgcgaccttccgccaaggtagatactgcgggctatgcaccaaagtctctgaggcagacatgtaagcgagctcttcacctatattcattcttttcctcctggacaggttacatttcccagtttcctttgcagttagttgtggctatatgacagaattctcatcaatggaaatgtacacagaagagaggtaagccactaccaggccaggcctataagacagcactttctacatgctttccccagacatagcaacccaaacatgaccacatcccttaagggaagatggagctgaaaataatggaaggaacttggaatgctagaatgctgaattaccacctgggagacagctacccactgacctggaatacctgtcctggactgttacatgagcaagaaatacacttctatttatgtatgagttacttcattatcagatatttattacagcagtttagctacctaagatctctctctgcctcagactgcttatctataaaatggaataacaccatctactccaaacattattgtaaggatgaaatgagacaatgctgaaaagtgtttaccataatatctgccacacaataagtaccccatatagtatttctgtattagtaagttacatgagagattttcttcttttaatacatctgcatttataaacattttactttaacctcaacttccccagcactgctctaccattttctgaatgtcattatgagagaaataaaactaatttctagggccaggcatggtggctcacacctataatcccagcattttgggaggccaaggtgggaagactgctttgaggtcaggatttcaagaccaacctgggcaacacagtaagaccccatctctataaaaaaatgaagaaatcagagggtacagtggcacatgcctgtaatcccacgactcagaaaactgaggcaggaggatcgcttgaacccaagggatcaaggctacagtgagccatgatcacaccactgcattccagcctgggcacagagtgagaccctgtctctaaaaataaaaaatagggccaggcacagtggttgatgcctgtgatcccaacactttgggaggccaaggcaggtagatcacttgaggtcaggcgtttgagaccagcttggccgacatggcaaaaccctgtctctactaaaatacaaaaattagctgggcgtggtggtgcacgcctgcagtcccagctacttgggaggctgaggcaagacaatcacttgaacccaggaggcggaggttgcagtgagccaagatggcgccactgcactcaaacagaatgaaactctgtctcaaaaaaaataaaataaataaaaatttaaaaactaatttcttataatccagttgtgaatttaaccaatgtctgaaagaactattaaaagttaaaatgaatggaaaacagaataaagggttgaccagaacagatgtgattttctacttaaatcttttttttaaaccccaaaattcaaaactgctaatgttttttaatacgaatttctatctttgataaggcaatctgagtattacctttcaatccttcaataaaagtatcccaaacagaagggctattactgtaactaagcttgatactctccttcgctcttttcaag

SEQ ID NO: 26 - DNA, 3804 bp, Homo sapiens
  misc_feature (2122)..(2131): n is a, c, g, or t
ggcttctggctctgagtgaggtcctgctgcaaggtttcctagatgagccactgagactctaataagatccagtggaaataaccaggctctcgtcggaatataagtcccaagggaagctgtgccagtcttgtgggcgactgcctgacttctcctttcatttcagcaccatgaagcttctcacgggcctggttttctgctccttggtcctgggtgtcagcagccgaagcttcttttcgttccttggcgaggcttttgatggtaaggcttcagaaggtttgcaggatttctgaagagaaacatcaccctggacctgataaactggggaaaatgatgctttcggaaggctgcttttgaaccacagagttgctagtgtctgcgttgctgaggcctgccaggaactagggtttgctgggttgcctgtctcgagtctttcagagctgctgggaatatcccctttccccgtagtgcagcttctcaggatgtgttaagtggatggatcacatttcagaagccgctgcaaggtgtatcaaaaacacatctcctgagccgtaagggacggggcatccagtaacaacgcacacggggtatttttgggcttccttaagatttgagccgctgccttaggttgtgctgcccaatgtgcctggggagctgctaaacagattagagagtcgaggattgttgtcagttactcagagaaagaacaatcatcctttccaggagcacctgagctgtttgttttgcgtagaagatgcaaaataaggcctgcaatgggtataaaatgtccctcagcataaatcgcataggagtatgactaaggctgttgactcttctgtcttctttctccttcctccttcgatttcctagttggataatgtacagggctctttagcctcgctctgtcaggggctcccttcctggtttgttctgtttccattcttccttctccagccttcttgacaagagctgggaactaacgtgcctcaagcccccacaaggaccacagcattttctcatttagtttcagaatgactctgtgacgcaatcttcctctcttggaaggtgagaaagctgatcttggaaggtgagaaagctgagacttagagcagctgaagccaatgcccagggacttactgccagtcagcaggtggcagggcagaggtttgagcccggctgtgcttgaggtcagggctcttgccaggtagacgcatcactgaccacctcctagaggttgatggttatgaatctcaggcacaccttggcatcacctgaaatacccatgccttcaactccccagcagagtctgcagaaactggcctggggtgtggcctgggcactgggactttcagtttctctctgggtgattagaaagtgcagccaaggctcacgcctgtaattccagcactttgggaggccaaggtggatgaatcacttgaggtcatgagttccggagcagcctggccaacatggtgaaaccccgtctctactaaaaatactaaaatgtagccaggcgtggtggcaggcacctgtaatcccagctactcaggaggctgaagcacgagaatcacttgaacccgagaagcagaggttgcagtgactagagatcgcaccagtgtcctccaacctgggtgacagagcgagactccatctaaaaaaaatgaaaaagaaagtgcagccaaggcagagcaccactgccctattgcttcctcaagcaacccacagcatcagtacagcctactaagaaagtatttagggacttttatgctcctaacagtcactggaactcacgtcacaatgacgtgtattccatttgcaagaatatatactttaggtcggggtgcggtggctcacgcctgtaatcccagcactttgggaggccaaggcagggggatcacgaggtcaggagttcgagaccagcctgaccaacatggtgaaatccccgtctctactaaaaatacaaaaattagccaggcgtgatggcgcatgcctgtaatctcagctactcaggaggctgaggcagaagaatctcttgaacctgggaggtggaggttgcgatgagctgagatagcaccactgcactccagcctgggcgacagagcaagactctgtctaaaaaaaaaannnnnnnnnnaaaaaaaaaaaaaaaaaaaaaaaaaaaaaaaagaatataaactttagtagtcagggcagaagtactctgtgtctgccacctttctcagcatcagtattccatgtcactacctcattcatacacactcctggatcttatcataggcagcttcattctatagcagtggctcttcaccagggcacttgaagaagccaactaggataaaggaatgtgcttctcaacccatggtatccaaggctgctatgatcacaggctgaaagcttgaagtcagtggaagatttgtccttcctcattcccctctaaggtgttgttggagtctttatgttctcctgatgtcccttctgcctttcctttcctttccaggggctcgggacatgtggagagcctactctgacatgagagaagccaattacatcggctcagacaaatacttccatgctcgggggaactatgatgctgccaaaaggggacctgggggtgcctgggctgcagaagtgatcaggtaactggagctcctgggacgttagggctgggtgagcagagcttgcctgccttggacagtcaggagggagacgagctccttgtggagaagttagaggctgcggcccctcctcctcttgccctctctctgcctctgtgctcagtgtgaggtctgagtggatggtaggagtgagtgattcctcatcctccctctctgggtgctgttcatccagcctaggggtgcccagcctggctgaatggggtggtgcccagtgttttcatccctccttccttggcctttctgggctcctctctgagccctcccttggaacagggagaatgggagggtgggctattgctcactggcctgattattaatctccttcttgcctgccttgattacagcgatgccagagagaatatccagagattctttggccatggtgcggaggactcgctggctgatcaggctgccaatgaatggggcaggagtggcaaagaccccaatcacttccgacctgctggcctgcctgagaaatactgagcttcctcttcactctgctctcaggagatctggctgtgaggccctcagggcagggatacaaagcggggagagggtacacaatgggtatctaataaatacttaagaggtggaatttgtggaaactgggtgttatactttgtggtatagactgcctgtttagtatgaaggggcgatccatgcacatctaagtgaacgtggaggctgggtgggtgggagacgactcctgggcacacagggcatcctgggcatccctgaggcaaggacatgatgagttcagtggccacccccacaggatcccaggggcttcagcagatcccaccccttaccccatgtgagcagctgcccagtgagtctgtaggaacccgagccacattcccagtgagttcaactgcaccccggcacgttttgctagcacctcaatggagagctccttgcttgcagctttggcttgtggcacccagcaaaagcttcctgccacccagtggctacagccacacactctccagcaagatttaatctcagccttgtgaggagccctttcccaaatttatttctttctgtgttttttatcccttagtagctaatctcatgttagccattaataactctctatgttaaacccttccttttgtatctgcggctacattga

SEQ ID NO: 27 - DNA, 3804 bp, Homo sapiens
gtataaatgcagaggtgcagtaactgggcttttcaggatatccagatggagttgtggtgttgttttgcttgtggtttttaacgttaacttttttttcccctttattttaagagaagcacaaaatgaacaaactagtgagcccagcaacatggatggaaattccggagatgcagactgctttcagccagcagtcaaaagggtatgggcaaaaaaatatgaaccatttggggctcaagtttctccaaatactttatgtgactgcaagtactgtatacgcttatttcctgtgactcagttcttctaactaagatgttaagcatttggcttaaagtgtatagcattacaaagagtatttccccagctttggcttgccagccaactttccattgactctagcctgttagccatttttattgttttttgtttgtttgtttgtttgttttcctcacatgtacacatacatacagattgttcttatatgtgattttgttctctgggaataaaatcttcattcaacagaggcaatatgacagaaaaaccgaagtttcatgtatatgatttttcaaagaaagtgaattggccctcatgttaaacctagcatttcagagctgaaagtgtcttctcattaaatattgaagaaatcatttgagggtgtggagaaggatggacagaattagctgcttgtgtatttattcttctcctgcaactttgccacgctattttgtacctcccttcctaattatgataaagctttcttagagagcagtcaggcaatgtgtattaaatgtttaaagctttacacccttagttctacttgtggacatttatttcttaagaaagatgtatactaagatttagatagaaatattcattacagtatcataataaagacagtagcaaggattctgttatctgtgttgcattaatacaatagagattgatgcaactgttcattattttgaaagcattaatgataatattgcatcaaagagttcactgaacagattgtacagtacagttttacacacaaaaaaaatagtttgtgagctttaaaagggccttcaaatgaatatgctaaacggttatctttcaataaagagagtatgggtaagtcttaatttctttcatttatttcagtaatttaatgtttttgttgttgttattgtttgtttttttgagacagagtcttgctctgtcacccaggctggagtgcagtggtgcaatctcagctcactgcaatctcggctcactgcaacgtctgcctcctggattcaagcaattcttctgcctcagcctccggagtagctgggattacaggcgtgcaccaccatacctagctaatttttgtatttttagtagagacggagttttgccatattggccaggctggtgttgaactcctggcctcatgtgatccgcccatctcagcctcccaaagtgctggggttacaggcatgagccactgtgccagcctatttcagtaacttaatgtttttacaggcatgtattacctataaaattaataaagccagtgaggtatttcttttttgaactaaagcaaagctaataataagttatagagaagttagagaagaaatctattaagtgatactttctttgtatactgttgggctgagtacccttgattcttggtggtgaacaagttatcagaaatttcttggccaggagccgtggctcacacctgtagtcccagcactttgggagtccaaggtgggtggatcacttgaggtcagaatttctagatcagcctggccagcatggtgaaaccctgtctctattaaaaatacagaaattagccaggcatggtgacgtgcgcctgtaattccagctacctgggaggctgaggcagcaaaatcacttgaacctggcaggcggagttcgcagtgagctgggatcgcgtcgctgcactccagcctggatgacagagcaagactccatctcaaagaaaaaataaaaaagaaatttatttacttgtgtgaatttttacaatacagatgcttctcgacttaaatggggctacatcccaataaactcataagttgcaaatactgtaaatcaaaaatgcattgaatacacctaatgtatggaacaccatagtttagcctatcctactttaaatgtgttccgaacacttagattagcctgtagttgggcagcattacctactataaagtgtattttctaataaaatgttgaatatctcatgtaactcattgaatactgaaagtgaaaaacaatgtatgggtactcaaaatatggtttctctactgaatgtgaatcactttgacaccatcataaagttgaaaaattccaagtcaaaccattgtaagtcaggggctatcagtattcagtggtaaatgctggctctaactattcttccaagtcagtggttgactgctgtttattctataaagggttacaatttatagattctctcacttgtagaatgagagattcagaattaatagcagacagagtccctaccttgatggagctttcatttaagtgtgaaagtcaggtgacctaacaaggccttggcataagtttaggatttggattgttatgggagcttgggtagggacatgtcataggtaaggcaacagcaggggtagagataagcttgacatatgtcaaaaatcatgaagacatcagtaatccttgaagttggctgaaaggtatagagttgagaaagtagttaaaaaaaaaaaagtcaggctgagtctaggtaaggatgtgtttctctgaggtcagatttgttcctgtaccataaagggactatttagaatcttaaagctggagcaatttaaaacgttaagttttcagattgaggtcagatttgtgacttcatgtgaggtcagatttgttcctgtaccataaagggactatttagaatcttaaagctggagcaatttaaaacgttaagttttcagattgacgttttttgaggtatagttaataacctgaatgttctgattctagtcttggtagtcaataagagttgaccagatgaatttcatagctttgtagaggatgaaatatttcaaggctgatttgcacaaatgtttacatagatcatgtatctttcataagtaatatgtttgtattattacaaggctgtaaaaatttaagcaggttgttaatagcacagggggtaacagattaataaaattaatgaataaaattactaaaagagtccagaagtaaacccaaatacgtggaggaattaagcatatgtatgatacacatgacattttaaaaatcagtgggaaaaggtaaattattttacaaatggtgttagaagcactgattgataattttgttaaaagaaacttagattccctattttactcctaatccaaaataaattctgagtggatctaagattaagcaaaaattaagccggaagctgagcatggtagcatgtgtctgtaatctccgcaatttaggagactgagtttggctggggaggtggtgatatgcgcctagaaaaaaaaaattttttaagccacagatgtataagcaaaaagcgggcaaagaggcggaatttttttttttttttttgatgaagtctcacttgtcgcccaggctggaacgcagtggcgtgatctcagctcactgcaacctctgcctcccgggttcaagcgattctcctgcctcagcctcccaagtagctgggattacaggcacctgccgaggagaggatttttttataattaaaacaaaacaaaacaaaaaaacaccaaactggaagataaagtatttacaacatgtaaaagactgttt

SEQ ID NO: 28 - protein, 122 aa, Homo sapiens
MKLLTGLVFCSLVLGVSSRSFFSFLGEAFDGARDMWRAYSDMREANYIGSDKYFHARGNYDAAKRGPGGAWAAEVISDARENIQRFFGHGAEDSLADQAANEWGRSGKDPNHFRPAGLPEKY

SEQ ID NO: 29 - protein, 122 aa, Homo sapiens; identical to SEQ ID NO: 28

SEQ ID NO: 30 - protein, 122 aa, Homo sapiens; identical to SEQ ID NO: 28

SEQ ID NO: 31 - DNA, 5687 bp, Homo sapiens
ctctctggttgcccttaacattttttccttcatttcaactttggtgggtctgatgattatgtgtcttggggttgctcttctcgaggagtatcttagtagtattctctgtatttcctgaatttgaatgttggcctgtctttctaggttggggaagttctcctggataatatcctgaagagtatttttcaacttggttctattctccttgttactttcaggtacaccaatcaaacgtagatttggtcttgtcacatagtcccatatttcttggaggttttattcgttcctttttattcttttttctctagttttgtcttctcgctttatttcactaagttgatcttcaatctctgatatccttgcttctgcttgattgattcagctatcccccgctcgatattacaaaccatgtcacgaggcgtggacaccccccatgatatggggagtattatcacccccctcttcccccactggatattacaaaccatgtcatagggaggtggacatcccccacaatatgaggagtaatatcacacccctttccccgcagtggatattatgaaccatgtcacaggcggttaaacacccccaacgatatggggagtaatatcacactcctctcccccctggatattacgaaccatgtcatggggggtggacaccctttgcaatatggggagtaaaatcacccccctctcccccaactggatattatgaaccatgtcacagtgggggaaaaatcctctgtgatatgcagagtaatatcaccccactctcaccacctggatattacgaaccatgtcacaggggggtggacaccccccaagatgggggagtaatatcacctcactctctgccaccagatattacaaactgtgtcacaggggggtgaacaacccccacaatatggggagcactatcacccccctcccccagggtattatgatccatgtcacaggggggtggataccacccactatatggggagtaatatcacctttctctcccgccctggtttttatgaaccgtgtcacaggggggtggacaccccttgcgatatggggagtaatatcacccccctctccaccatctggatattacgaaccatgtcacaggggggtggacacccctgcgatatggggaggaatatgcccctctccccacctggatattacaaatcatgtcacgggggacggacatcccccacaatatggggagtaatatcaccacactctcccctgctggatattacgaaccatatcacaggcggctggagacacaaggcattaacaatatttcgagtaatattatctttccctttgaacattatgaacaatatgacagaggggtgtacacctcctgcgatattgggagtaatgtcatcccctcccccactggatattaggaaccatattactgggggatgtattcccccttctagattgggaggaagatcatacttgccctccctgaatatttgaaacaatatcataggggtttgtacacttttacgatattgggagtaatatcatcctttctccccctggaaattaggaacaatatcacaggggtggtgtacacccctgcaatatttagggtaatattattgtcttctcccctcgatattaggaacaatattacaaggacggtgtaaagtacctgccaaattgggaaaaatactatcctctccctcttgtatattagaaacaataacacagggggaatgtacacccactgccatattgggagtaatatcatactcgccccatcccccagatattaggaacaatatcacagcaggggtgtacacttttacgatattgggagtaatatcatactctctccccctggaaattaggaataatatcacagagatggtgtagaccctctgcaatacttaggataatattatcatctcccccctcgatattaggaacaatattacggggagtgtaaattacctgccaaattggaggtaatcctctcctctctctccctgtattttagaaaatataacacacaggaaatgtacaacactgcgatattcggagtaatatcttcttctccccacctggatattaggaacaataacacggacggggcgtacacccctcgcgatattgaatgtaatgtcatcctctccctccctttatattacgaacaatatcacaggggggtgtacaacccctgcaatattggaagtagtatcatccattctcccatgaatattaggaacaatatcacaggggtagagtacaccctctgcaatttcgggagtaacatcatcctctcgttccctggatattataaacaacaccacgggggggtgggggtgtacacacccttcgatattgggagtaatataatcctttccctccctatatattagaagcaatatcacaggggttggtgtaaacttcttgcgatatggggattaatatcacccccctctcctgccctggatattatgaaccatatcacagggaggtggacacactttgcgatatggggagtaatatcacgcccctctcccccccgatattacgaaccatatcacaagggagtggaccccccccacgatatggggagtaatatcacccccctctcccgccctggatattacgaaccatatcacagggggatggacaccccccgcgatgcggggagtaatgtcacccccttctgccccctaggatattacgaaccatatcatggacaccctccacgatattggaaataatatcatcctctcccccttggatattaggaacaatatcacagggggttgtacacctcctatgatattggaagtaatatcatcctctccctcctggatattagcaacaatatcacagggagtgtgtacaaccccagcgatatttggagtaatatcaccctctcaccccatggatatgagaaacaatatcacaggggaggtgtacatcccacgtgatattgtgtgtaatatcattcttccccaacccctgcaatattgtggtgtaatataattctctcccttcctggacattatgaacaatatcactactaggtgatacattaggagtaatgtatccataggatattatgaggaatatcacagggtgtacacccactgtgatattagaggtaatatctccctaaaatattaagaagaatatcttacacccactgtgactttagaagtaatatctccctaaaacgttacaaataacatcgcagggtgtacactcacagtgatattaggagtaatatctccctagaatattacaaatacacatggtgtaaacccactgtgactttagaagaactatctccctaaaataatacaaaaatatcgcagtgtataccataatatcccctagaatatcataaataatatcacagggtgtacacccactgtgataataggaataataccaccccaggatattatgaataatgtcacaggctgtacacccactatgacattaggagtaatatctccctaggacactatgaataacatcacagattttacacccatggtgtgcacccactatgatattaggagtaatatctgcacaggatataacaaataatagtacagggtgtacacatatgatatacacccactgtgatattaggagaaatatatccctaggatattatgaataacctctcagagtacacacacatggtatacaccctctgtggcattaggaacaataactttctaaaacattacgaataacatcacagaatgtacacacatggtttacacccactgtgacaggtgcaatatctcccttggatattatgaataacaacaaactatcactgtcatattaggagtaatttctccctagaatattacaaataacatcacagggtgttcatttatggtgcacacccactgtgatattaggagtaatatctccctaggatattacttttcatataaaagtgtgtacatccactgtgatattgggaaaaatatttctctaggatattatgaataatatcacagagcgtacacccactgtgatattaggagtaataattccctgggttattatgaataatatcacaggatgtacaaccactgtgatattaggagcaatatcttcctaggatattacaaataatatcacagggtgtacacccactgtgatattaaagtaatttttaggttattgtgaataatatcaccaagtgtacaaacatggtgtacactcactgtgatatcaggagtaatatctcagtaaaatattatgaataatatcacagggtatacacccactgtgatattagcagtagtatctttgtaggatattacaaataatatcacagggtgtatgcccactatgacattagaagcaatatctccctaggatatcaaaaataatatcacagggtgtacaacttctacatcccaggttctaagggattctcctgcttcagcctcctgagtggctgggattacagatgcccaccaccacacctggctaatttcgtattttcagtagagatggggtatcaccatgctggtcaggctggtctggaacttctgacctcaggtgatccaccagcctcggccttccaaagtgctgggaatacaggtgtgagccaacgtgcttggcagagagttatatattaaataaatctggaaacatagctcccatgtttgagtgtgcatttacttttatgaagaaattatgtcagaaaacctaaggatgataataaatatgaaaagtaactggcatgtaaaaaggtcttttgattaagaactataaggttcgatttcatttttagataacgtgatcctagctcttgtatagtgcttataaatattctacatcaaaggaatttgttgcacagtgtcagaataaaataaagtgtatttcactgcttcttaatttttaaattagactgagtttgttttcctagagagagaagaacattttttattttttctgaaaagagtaggccatattttactgagatcttagatttgttatatattaggttttggtcttctaacattctccagtggattttctctaaagtaggtatgcacagaaagagttgaatagcaaaaaagtaaatcatgtaataattctgagatttttgggtttgtcacaactgagaaatattgctgagggtgtatggtcctcaagtgtgaaaatgttccttgtgaattgcttgtatccgaaatatacacacaacattaagtcctggtttttatcttttattttttccaatccttttttcttctcaaggtgtccaagtcacacagagccacagaatctcacaggtgtctcagaattcctcctcctgggactctcagaggatccagaactgcagccactccttgctgggctgttcctatccatgtgcctggtcacgatgctggggaacctgctcatcatcctggccgtcagccctgactcccacctccacatccccatgtacttcttcctctccaacctgtccttgcctgacattggtttcaccttggccacggtccccaagatgattgtagacatgcaatcacatagcagagtcatctcccatgcaggctgtctgacacagatacctttctttgtcctttttgtatgtatagatgacatgctcctgactgtgatggcctatgactgatttgtggccatctgtcaccccctgcactacccagtcatcatgaatcctca

SEQ ID NO: 32 - DNA, 5687 bp, Homo sapiens
attgaattttatctcagagcccacatgaagcaggatcaaagtcagtacacatgaaaactagagcccaaagactataaagcatgaaataaggatttaagctaaccctatcttgtaaggggtttgtaaagcccagcttgcatctgagctacactagcaccaggacagccactcagtaatggggtttctcaaggttattgcttttcattcagttgaaatgagagtcatttcttacccttatgccctgtgagatttcactggaggttgttcactgaaacattttcatatcattgcatcaaccctcttgaactcactgtgcctgcccccagttcagtctgtgactcacaagtaccctgcagcaaaagaaatccaatagagggcaaatccctcaccttaccttcctttctaagacctttgatgttctcatgtgtcatttcataattgggattgtcaattagtcgcctcatctctggtcctcactttcctctctcccagccaaactcaaccttcagcccacacaatggaattcaacaaaatgaggtaacagttttctgtgtgagtcactctgggcaactctgttcacagagcactgtgaggtgagcagccagaacccaggcaagtgtttcagccatccaagaactggcaggcagcccaagagacactctcacctgatgacagactagcaggatgagtcctggaggaaatggttcccaacagctgcagaaggagtctcttggctcatgcacagcaatgctcttctcaattaaaaacgttgtcattattgacactgcagtgtaaaatccttttacactgtgctcacatttctacaggccttcacctgctctgcccattaaagacaagacccttccatgagatgatgacatctctaagttactgttccacccaaacagtcctatataatgaagagaaaaattttgctggccctcaaaaggcaaacacaaggagaaagatttccacaagctgtttctctttgctgagcacttagaggaaaactgtaagtggttggaagaaggctttgttttctacaagacttttagttattcctcagaaattttcctgcttattcccagaggaggtcatctcttagatgctgtcagtcagatagggattggcagccaagcagaggtgctcagagaggtttccaactaatgtggccagcggaaaactgccaaagaagcagggatccttaggacaaataaactggaagatattttggggataaaaataaatccttttgaaaatgaaagatggagagatgctgtatatacaaattgccctgttctgaacaatgttgtcactaggactggccctggagaccaatgatacaaaccaaaatgttctcagacatgctttgatggtctttttctccaaagttatctattctgtttccatttcattctcacaggacttgccatggggttctcataagatttcacattggtcataatccaggtggccctggactgcaacctctgagttggcaacatcagaataggaattacgaaaaaccaatttaaagttaaatacagacacaggcaaaagagagatgggttgtcgaagctagtgcctaggtggacactgcctcacatttttaattccagaagccatcagtactgagtgtcagatctcattagtcaaacacagtgatcaggaatcctgttttcctggaggatttccttgagggagggaccactcaagagtctgaaatatttcacgtcatagagtatggatctcaccccaacacccaatcagaaaatagggagaactggaaaccaaaattccccctcccgctgtggaaggatgaaaaccagagtgttggagttctgtcctgataatggagcagacagctaggcagcaatcaatgagggccagtacaggaattcagtgctaagtattgggtcataacagaagtagggaaggtattaatccagtgctatatgaggatcctgggacactggctcctagtaatctagttataactattagcaaaaaagaaaaaaaaaatcagtgatgtgaagagatggcctaaaggagctccagcaatatagctaagcagctggcaagtggtctgaggagcattgcaattccaggcctcctaaggtggcagtacgggcactggtaagacattctgctgtggtgaaactagtttaccatagaggattcacaattaaaataggcaaacaggaaatgcaagacagaggctaacaaagggttttttttttggtgggggggagttgtttgtttgtttgtttgttttctgagacggagtcttcctctgttgcccaggctggaatgcagtggcacgatctcagctcactacaacctctgcctcccaggttcaagcagttcttctgcctcagcctcccaggttcaagcagttcttctgcctcagcctcccaagtacctgggactatagctgtgtgccaccacattgactaatttttgtacttttagtacagactgggtttcaccatgttggccaggctggtgtcgaactcctgacctcaagtaatccccccgccttggcctcccaaagtgctggaattacaggcatgagccaccacacctggccagtttttggtaattcttaaagaactcaatgagcaacactcaaacaaccataaagactatagagctcatggttgaattttagatagctaaacagacaggagtttttgtaagttttgtaagtcttgctcatccttccctcttccatcctctatctcaactattctgtctaccattaaagcaccttagaccttgagtttggcaatgcaacaagtgtgtgctcaacacgaaataggtaattcaatagcaaagccctaaaacagcctggcttgattatttctcagggcatgcagttcctttgaagcaggatcattttaataataataataatagaaataataatagaaattgaagacaattatttcacaatttccatacacctaagagctatacatatgaatgataatgcataattgtaaagcatgcatattacaggtaataaatatgttagctaattataaacaatgcccattttcatatagtttatccttgccaaataaaactgtaaaaaaaagacacctttcaaatgctgctaaggagtaatacctgaatgaggttgatttaatggagtcttagttcctgcatgtgttctaattgaatagactatgtagtaattcccttacatacccatccatgtccaagaacagtgaagatctttatttaatatgaattattgcagatgattagcacagtctagccaaaccattccagtaattgtttttacttgttatattaatatataaattctcaaaggatataacagtgatgttgggtgaatttcactgaatgatagctcaaacacctgaaatattgactaagaaaactaatttatcaatactgataatcaattttaatatgttaattgattgtaatacaggattctgtggttcaaaaaaaaagaacaagcaaaaaaactttcttccatttccaaataccaattaatagatctctacttccccttggatttcttcttaccacctaccacctccaatcttcattctttcctcacaaactaaacataaaagttacctacaaagcatagaatctgtgttaaaggatattcttgcttgttttaagtccaaaattaaacagctctgaattattaaaaagcacatgaattcaaatgtcctattctaataagaaaatggtttacatttctctatgttcaaggaaaaaaatagtcaagggtgtacaagtggggtaaaaattatttccagtaggttatgtgatttaagttatagaaacgaaccaggcaattcaattaaatgtcatggaaagtaggttttttcttttcctctttttttctaatatgtacactttgtgagaagataaatccatagtgtgataatttgtccactgggtccatcagacactggagacagcttcctaagaattataaggcttctaaaggcttctaaagcctaaattgcctagagcattttgtgtgccaggcactttgctaggtgccctagggatgcaagaagtataaatgttttatgagaatacaggctggaaatgtattcttgattattcctgtggaatttctaggcagaaaagagtctaatggggtataggtatattttctcaacacaattttctgagcctttaccagatgcagttctatggtttgaatgtgtccctcagagtttgtgtgttggaaacttaatccccaatgcaataatgttggtgaggcctaatgaaagcctaataatgtaggtgaggcctaatgagagctgtttagaccatgaaggctcttccctcatggatggattaatgctgttatggtgggaatgggttcattattactggggtgggttcataataaaaagatgagtttggcctgctattctctctctttctcatcctctcttccaccatgggatgacacagcaagaaggcccctgcaagatgccctcccctcagtattggacttcacagcctccaggaccataagccaataaatttttgttcattataaatttcccagtctgtggtattctgttatagcaacactcaatttatgcattacttccagattcttatggctatacctacttctcacagtttgtattcacccctccttcaaccaagtacccttaacacagttcccatagtcacaaagccaggtcactgaagctgccctctctccaaccacacacatatagatcaaatgaccccagacatagagctgattgagaaggagggaccagtacgagctctgcttccccagcagcttcctggaaagaagaggcaatacaacccaacccaaaagtgcaagagaagtaacacctcatgggatgagcttaattaatcaatgggagaggacactagaagacactagaggatctcccttcctccctttctttcccacttcaccccctccagtctctgaaccatgagctatttcaaaggtgcagtaatgctatatttggcttctctgaagatatcctatgaggccaagtcatcagctttgttcattatctaagagtggtggccagctcaccagcacttcccatcatgtttgccctccctctttcccttgtgttacttcccattttcccttacttctgctttcttggcattaaattctactctgcaatgttaggatataagtttttgcctcagattctgttttctaggaaacccatgctaagacaacactggcagtggccctggaaaagtaaacctcatgatggatttggagttggattgttcactgatctgaaggacagaggactccacttaagtggtaagcagtgtagctatgaactctgccacgcaggcctcacaattactgaggcttcttttacctgtggttaactgggacacagaacagcaggaaattgagtgtagaggttatcaagtagctgcttcacttaattggtataattttatggagttaacctggtttagagtccagagaacattccacatagcctagaaagggtagttatttgtccttaccataatcaagtcatactttgaatatgagttttccttccctgttcagcaccacttctcttagacttaagaatgcctgatctgttgatattatgtcccatgtaacattgcctgagacaaagatatccatgtaccttaaa

SEQ ID NO: 33 - protein, 140 aa, Homo sapiens
MGFQKFSPFLALSILVLLQAGSLHAAPFRSALESSPADPATLSEDEARLLLAALVQDYVQMKASELEQEQEREGSSLDSPRSKRCGNLSTCMLGTYTQDFNKFHTFPQTAIGVGAPGKKRDMSSDLERDHRPHVSMPQNA

SEQ ID NO: 34 - protein, 128 aa, Homo sapiens
MGFQKFSPFLALSILVLLQAGSLHAAPFRSALESSPADPATLSEDEARLLLAALVQDYVQMKASELEQEQEREGSRIIAQKRACDTATCVTHRLAGLLSRSGGVVKNNFVPTNVGSKAFGRRRRDLQA

SEQ ID NO: 35 - protein, 141 aa, Homo sapiens
MGFQKFSPFLALSILVLLQAGSLHAAPFRSALESSPADPATLSEDEARLLLAALVQDYVQMKASELEQEQEREGSSLDSPRSKRCGNLSTCMLGTYTQDFNKFHTFPQTAIGVGAPGKKRDMSSDLERDHRPHVSMPQNAN

SEQ ID NO: 36 - protein, 116 aa, Homo sapiens
APFRSALESSPADPATLSEDEARLLLAALVQDYVQMKASELEQEQEREGSSLDSPRSKRCGNLSTCMLGTYTQDFNKFHTFPQTAIGVGAPGKKRDMSSDLERDHRPHVSMPQNAN

SEQ ID NO: 37 - protein, 187 aa, Homo sapiens
TSEETISTVQEKQQNISPLVRERGPQRVAAHITGTRGRSNTLSSPNSKNEKALGRKINSWESSRSGHSFLSNLHLRNGELVIHEKGFYYIYSQTYFRFQEEIKENTKNDKQMVQYIYKYTSYPDPILLMKSARNSCWSKDAEYGLYSIYQGGIFELKENDRIFVSVTNEHLIDMDHEASFFGAFLVG

SEQ ID NO: 38 - protein, 168 aa, Homo sapiens
VRERGPQRVAAHITGTRGRSNTLSSPNSKNEKALGRKINSWESSRSGHSFLSNLHLRNGELVIHEKGFYYIYSQTYFRFQEEIKENTKNDKQMVQYIYKYTSYPDPILLMKSARNSCWSKDAEYGLYSIYQGGIFELKENDRIFVSVTNEHLIDMDHEASFFGAFLVG